European Patent Specification EP 2 704 750 B1, published November 1, 2023. Title: TOLEROGENIC SYNTHETIC NANOCARRIERS FOR ANTIGEN-SPECIFIC DELETION OF T EFFECTOR CELLS. Applicant: Selecta Biosciences, Inc. Fraser, Christopher Kishimoto, Takashi Maldonado, Roberto. The sequence listing filed with the application follows.

SEQUENCE LISTING (944 sequences)

SEQ ID NO: 1 - protein, 18 aa, Artificial Sequence
  Homo sapiens Aggrecan core protein precursor epitope
AGMDMCSAGWLADRSVRY

SEQ ID NO: 2 - protein, 18 aa, Artificial Sequence
  Homo sapiens Aggrecan core protein precursor epitope
EDSEATLEVVVKGIVFHY

SEQ ID NO: 3 - protein, 18 aa, Artificial Sequence
  Homo sapiens Aggrecan core protein precursor epitope
SRVSKEKEVVLLVATEGR

SEQ ID NO: 4 - protein, 18 aa, Artificial Sequence
  Homo sapiens Aggrecan core protein precursor epitope
VVLLVATEGRVRVNSAYQ

SEQ ID NO: 5 - protein, 18 aa, Artificial Sequence
  Homo sapiens Aggrecan core protein precursor epitope
VVVKGIVFHYRAISTRYT

SEQ ID NO: 6 - protein, 9 aa, Artificial Sequence
  Homo sapiens alpha 2 type VI collagen isoform 2C2 precursor epitope
DRASFIKNL

SEQ ID NO: 7 - protein, 20 aa, Artificial Sequence
  Homo sapiens arrestin epitope
ASSTIIKEGIDRTVLGILVS

SEQ ID NO: 8 - protein, 20 aa, Artificial Sequence
  Homo sapiens arrestin epitope
ASTPTKLQESLLKKLGSNTY

SEQ ID NO: 9 - protein, 20 aa, Artificial Sequence
  Homo sapiens arrestin epitope
DRTVLGILVSYQIKVKLTVS

SEQ ID NO: 10 - protein, 20 aa, Artificial Sequence
  Homo sapiens arrestin epitope
EFARHNLKDAGEAEEGKRDK

SEQ ID NO: 11 - protein, 20 aa, Artificial Sequence
  Homo sapiens arrestin epitope
EPNHVIFKKISRDKSVTIYL

SEQ ID NO: 12 - protein, 20 aa, Artificial Sequence
  Homo sapiens arrestin epitope
FEVKAFATDSTDAEEDKIPK

SEQ ID NO: 13 - protein, 20 aa, Artificial Sequence
  Homo sapiens arrestin epitope
GFLGELTSSEVATEVPFRLM

SEQ ID NO: 14 - protein, 20 aa, Artificial Sequence
  Homo sapiens arrestin epitope
GKIKHEDTNLASSTIIKEGI

SEQ ID NO: 15 - protein, 20 aa, Artificial Sequence
  Homo sapiens arrestin epitope
GNRDYIDHVSQVQPVDGVVL

SEQ ID NO: 16 - protein, 20 aa, Artificial Sequence
  Homo sapiens arrestin epitope
KPVAMEEAQEKVPPNSTLTK

SEQ ID NO: 17 - protein, 20 aa, Artificial Sequence
  Homo sapiens arrestin epitope
KVPPNSTLTKTLTLLPLLAN

SEQ ID NO: 18 - protein, 20 aa, Artificial Sequence
  Homo sapiens arrestin epitope
LLKKLGSNTYPFLLTFPDYL

SEQ ID NO: 19 - protein, 20 aa, Artificial Sequence
  Homo sapiens arrestin epitope
LTFRRDLYFSRVQVYPPVGA

SEQ ID NO: 20 - protein, 20 aa, Artificial Sequence
  Homo sapiens arrestin epitope
MAASGKTSKSEPNHVIFKKI

SEQ ID NO: 21 - protein, 20 aa, Artificial Sequence
  Homo sapiens arrestin epitope
NRERRGIALDGKIKHEDTNL

SEQ ID NO: 22 - protein, 20 aa, Artificial Sequence
  Homo sapiens arrestin epitope
PCSVMLQPAPQDSGKSCGVD

SEQ ID NO: 23 - protein, 20 aa, Artificial Sequence
  Homo sapiens arrestin epitope
PFLLTFPDYLPCSVMLQPAP

SEQ ID NO: 24 - protein, 20 aa, Artificial Sequence
  Homo sapiens arrestin epitope
QDSGKSCGVDFEVKAFATDS

SEQ ID NO: 25 - protein, 20 aa, Artificial Sequence
  Homo sapiens arrestin epitope
QVQPVDGVVLVDPDLVKGKK

SEQ ID NO: 26 - protein, 20 aa, Artificial Sequence
  Homo sapiens arrestin epitope
RVQVYPPVGAASTPTKLQES

SEQ ID NO: 27 - protein, 20 aa, Artificial Sequence
  Homo sapiens arrestin epitope
SRDKSVTIYLGNRDYIDHVS

SEQ ID NO: 28 - protein, 20 aa, Artificial Sequence
  Homo sapiens arrestin epitope
TLTLLPLLANNRERRGIALD

SEQ ID NO: 29 - protein, 20 aa, Artificial Sequence
  Homo sapiens arrestin epitope
VATEVPFRLMHPQPEDPAKE

SEQ ID NO: 30 - protein, 20 aa, Artificial Sequence
  Homo sapiens arrestin epitope
VDPDLVKGKKVYVTLTCAFR

SEQ ID NO: 31 - protein, 20 aa, Artificial Sequence
  Homo sapiens arrestin epitope
VVLYSSDYYVKPVAMEEAQE

SEQ ID NO: 32 - protein, 20 aa, Artificial Sequence
  Homo sapiens arrestin epitope
YQIKVKLTVSGFLGELTSSE

SEQ ID NO: 33 - protein, 9 aa, Artificial Sequence
  Homo sapiens Chain B, Structure Of Insulin epitope
ALYLVCGER

SEQ ID NO: 34 - protein, 10 aa, Artificial Sequence
  Homo sapiens Chain B, Structure Of Insulin epitope
SHLVEALYLV

SEQ ID NO: 35 - protein, 9 aa, Artificial Sequence
  Homo sapiens chaperonin (HSP60) epitope
QMRPVSRVL

SEQ ID NO: 36 - protein, 9 aa, Artificial Sequence
  Homo sapiens Collagen alpha-3(IV) chain epitope
GSPATWTTR

SEQ ID NO: 37 - protein, 9 aa, Artificial Sequence
  Homo sapiens collagen, type II, alpha 1 isoform 1 precursor epitope
ARGQPGVMG

SEQ ID NO: 38 - protein, 9 aa, Artificial Sequence
  Homo sapiens DNA topoisomerase 1 epitope
KMLDHEYTT

SEQ ID NO: 39 - protein, 9 aa, Artificial Sequence
  Homo sapiens ezrin epitope
EYTAKIALL

SEQ ID NO: 40 - protein, 10 aa, Artificial Sequence
  Homo sapiens ezrin epitope
LNIYEKDDKL

SEQ ID NO: 41 - protein, 9 aa, Artificial Sequence
  Homo sapiens glial fibrillary acidic protein isoform 2 epitope
NLAQDLATV

SEQ ID NO: 42 - protein, 9 aa, Artificial Sequence
  Homo sapiens glial fibrillary acidic protein isoform 2 epitope
QLARQQVHV

SEQ ID NO: 43 - protein, 9 aa, Artificial Sequence
  Homo sapiens glucagon receptor epitope
RRRWHRWRL

SEQ ID NO: 44 - protein, 9 aa, Artificial Sequence
  Homo sapiens glucose-6-phosphatase, catalytic, related epitope
FLWSVFWLI

SEQ ID NO: 45 - protein, 15 aa, Artificial Sequence
  Homo sapiens Glutamate decarboxylase 1 epitope
NMFTYEIAPVFVLME

SEQ ID NO: 46 - protein, 13 aa, Artificial Sequence
  Homo sapiens Glutamate decarboxylase 2 epitope
IAFTSEHSHFSLK

SEQ ID NO: 47 - protein, 13 aa, Artificial Sequence
  Homo sapiens Glutamate decarboxylase 2 epitope
NFFRMVISNPAAT

SEQ ID NO: 48 - protein, 9 aa, Artificial Sequence
  Homo sapiens Glutamate decarboxylase 2 epitope
FLQDVMNIL

SEQ ID NO: 49 - protein, 9 aa, Artificial Sequence
  Homo sapiens Glutamate decarboxylase 2 epitope
LLQEYNWEL

SEQ ID NO: 50 - protein, 10 aa, Artificial Sequence
  Homo sapiens Glutamate decarboxylase 2 epitope
RMMEYGTTMV

SEQ ID NO: 51 - protein, 10 aa, Artificial Sequence
  Homo sapiens Glutamate decarboxylase 2 epitope
VMNILLQYVV

SEQ ID NO: 52 - protein, 11 aa, Artificial Sequence
  Homo sapiens Glutamate decarboxylase 2 epitope
AFTSEHSHFSL

SEQ ID NO: 53 - protein, 12 aa, Artificial Sequence
  Homo sapiens Glutamate decarboxylase 2 epitope
AFTSEHSHFSLK

SEQ ID NO: 54 - protein, 11 aa, Artificial Sequence
  Homo sapiens Glutamate decarboxylase 2 epitope
FKMFPEVKEKG

SEQ ID NO: 55 - protein, 10 aa, Artificial Sequence
  Homo sapiens Glutamate decarboxylase 2 epitope
FTSEHSHFSL

SEQ ID NO: 56 - protein, 15 aa, Artificial Sequence
  Homo sapiens Glutamate decarboxylase 2 epitope
MIARFKMFPEVKEKG

SEQ ID NO: 57 - protein, 9 aa, Artificial Sequence
  Homo sapiens Glutamate decarboxylase 2 epitope
RFKMFPEVK

SEQ ID NO: 58 - protein, 10 aa, Artificial Sequence
  Homo sapiens Glutamate decarboxylase 2 epitope
RFKMFPEVKE

SEQ ID NO: 59 - protein, 11 aa, Artificial Sequence
  Homo sapiens Glutamate decarboxylase 2 epitope
RFKMFPEVKEK

SEQ ID NO: 60 - protein, 9 aa, Artificial Sequence
  Homo sapiens Glutamate decarboxylase 2 epitope
TSEHSHFSL

SEQ ID NO: 61 - protein, 9 aa, Artificial Sequence
  Homo sapiens Glutamate decarboxylase 2 epitope
VMNILLQYV

SEQ ID NO: 62 - protein, 9 aa, Artificial Sequence
  Homo sapiens Glutamate decarboxylase 2 epitope
ELAEYLYNI

SEQ ID NO: 63 - protein, 9 aa, Artificial Sequence
  Homo sapiens Glutamate decarboxylase 2 epitope
ILMHCQTTL

SEQ ID NO: 64 - protein, 11 aa, Artificial Sequence
  Homo sapiens heat shock 27kDa protein 1 epitope
QLSSGVSEIRH

SEQ ID NO: 65 - protein, 9 aa, Artificial Sequence
  Homo sapiens HLA class I histocompatibility antigen, B-27 alpha chain precursor epitope
LRRYLENGK

SEQ ID NO: 66 - protein, 9 aa, Artificial Sequence
  Homo sapiens HLA class I histocompatibility antigen, B-7 alpha chain precursor epitope
VMAPRTVLL

SEQ ID NO: 67 - protein, 14 aa, Artificial Sequence
  Homo sapiens HLA class I histocompatibility antigen, B-7 alpha chain precursor epitope
ALNEDLRSWTAADT

SEQ ID NO: 68 - protein, 14 aa, Artificial Sequence
  Homo sapiens HLA-B27 epitope
ALNEDLSSWTAADT

SEQ ID NO: 69 - protein, 10 aa, Artificial Sequence
  Homo sapiens HLA-B27 epitope
LLRGYHQDAY

SEQ ID NO: 70 - protein, 15 aa, Artificial Sequence
  Homo sapiens HLA-B27 epitope
RVAEQLRAYLEGECV

SEQ ID NO: 71 - protein, 13 aa, Artificial Sequence
  Homo sapiens HLA-B27 epitope
WDRETQICKAKAQ

SEQ ID NO: 72 - protein, 11 aa, Artificial Sequence
  Homo sapiens insulin epitope
ALWGPDPAAAF

SEQ ID NO: 73 - protein, 10 aa, Artificial Sequence
  Homo sapiens insulin epitope
LALWGPDPAA

SEQ ID NO: 74 - protein, 11 aa, Artificial Sequence
  Homo sapiens insulin epitope
RLLPLLALLAL

SEQ ID NO: 75 - protein, 9 aa, Artificial Sequence
  Homo sapiens Insulin precursor epitope
ALWMRLLPL

SEQ ID NO: 76 - protein, 9 aa, Artificial Sequence
  Homo sapiens Insulin precursor epitope
HLVEALYLV

SEQ ID NO: 77 - protein, 10 aa, Artificial Sequence
  Homo sapiens Insulin precursor epitope
SLQKRGIVEQ

SEQ ID NO: 78 - protein, 9 aa, Artificial Sequence
  Homo sapiens Insulin precursor epitope
SLQPLALEG

SEQ ID NO: 79 - protein, 9 aa, Artificial Sequence
  Homo sapiens Insulin precursor epitope
SLYQLENYC

SEQ ID NO: 80 - protein, 10 aa, Artificial Sequence
  Homo sapiens Insulin precursor epitope
VCGERGFFYT

SEQ ID NO: 81 - protein, 8 aa, Artificial Sequence
  Homo sapiens Insulin precursor epitope
WGPDPAAA

SEQ ID NO: 82 - protein, 9 aa, Artificial Sequence
  Homo sapiens Insulin precursor epitope
FYTPKTRRE

SEQ ID NO: 83 - protein, 8 aa, Artificial Sequence
  Homo sapiens Insulin precursor epitope
GERGFFYT

SEQ ID NO: 84 - protein, 9 aa, Artificial Sequence
  Homo sapiens Insulin precursor epitope
ERGFFYTPK

SEQ ID NO: 85 - protein, 10 aa, Artificial Sequence
  Homo sapiens Insulin precursor epitope
LCGSHLVEAL

SEQ ID NO: 86 - protein, 10 aa, Artificial Sequence
  Homo sapiens Insulin precursor epitope
LVCGERGFFY

SEQ ID NO: 87 - protein, 10 aa, Artificial Sequence
  Homo sapiens Insulin precursor epitope
LYLVCGERGF

SEQ ID NO: 88 - protein, 9 aa, Artificial Sequence
  Homo sapiens Islet amyloid polypeptide precursor epitope
FLIVLSVAL

SEQ ID NO: 89 - protein, 9 aa, Artificial Sequence
  Homo sapiens Islet amyloid polypeptide precursor epitope
KLQVFLIVL

SEQ ID NO: 90 - protein, 9 aa, Artificial Sequence
  Homo sapiens islet-specific glucose-6-phosphatase-related protein epitope
FLWSVFMLI

SEQ ID NO: 91 - protein, 9 aa, Artificial Sequence
  Homo sapiens islet-specific glucose-6-phosphatase-related protein isoform 1 epitope
FLFAVGFYL

SEQ ID NO: 92 - protein, 9 aa, Artificial Sequence
  Homo sapiens islet-specific glucose-6-phosphatase-related protein isoform 1 epitope
LNIDLLWSV

SEQ ID NO: 93 - protein, 9 aa, Artificial Sequence
  Homo sapiens islet-specific glucose-6-phosphatase-related protein isoform 1 epitope
VLFGLGFAI

SEQ ID NO: 94 - protein, 9 aa, Artificial Sequence
  Homo sapiens islet-specific glucose-6-phosphatase-related protein isoform 1 epitope
NLFLFLFAV

SEQ ID NO: 95 - protein, 9 aa, Artificial Sequence
  Homo sapiens islet-specific glucose-6-phosphatase-related protein isoform 1 epitope
YLLLRVLNI

SEQ ID NO: 96 - protein, 9 aa, Artificial Sequence
  Homo sapiens keratin 6C epitope
ALQKAKQDL

SEQ ID NO: 97 - protein, 9 aa, Artificial Sequence
  Homo sapiens keratin 6C epitope
DAKNKLEGL

SEQ ID NO: 98 - protein, 9 aa, Artificial Sequence
  Homo sapiens keratin 6C epitope
GASGVGSGL

SEQ ID NO: 99 - protein, 9 aa, Artificial Sequence
  Homo sapiens keratin 6C epitope
KAKQDLARL

SEQ ID NO: 100 - protein, 9 aa, Artificial Sequence
  Homo sapiens keratin 6C epitope
KLEGLEDAL

SEQ ID NO: 101 - protein, 9 aa, Artificial Sequence
  Homo sapiens keratin 6C epitope
NMQDLVEDL

SEQ ID NO: 102 - protein, 9 aa, Artificial Sequence
  Homo sapiens keratin 6C epitope
RLLKEYQEL

SEQ ID NO: 103 - protein, 9 aa, Artificial Sequence
  Homo sapiens keratin 6C epitope
WYQTKYEEL

SEQ ID NO: 104 - protein, 20 aa, Artificial Sequence
  Homo sapiens Keratin, type I cytoskeletal 17 (Cytokeratin 17) (K17) (CK 17) (Version 2) epitope
LRRVLDELTLARTDLEMQIE

SEQ ID NO: 105 - protein, 9 aa, Artificial Sequence
  Homo sapiens Keratin, type I cytoskeletal 17 (Cytokeratin 17) (K17) (CK 17) (Version 2) epitope
ALEEANADL

SEQ ID NO: 106 - protein, 9 aa, Artificial Sequence
  Homo sapiens Keratin, type I cytoskeletal 17 (Cytokeratin 17) (K17) (CK 17) (Version 2) epitope
ANADLEVKI

SEQ ID NO: 107 - protein, 9 aa, Artificial Sequence
  Homo sapiens Keratin, type I cytoskeletal 17 (Cytokeratin 17) (K17) (CK 17) (Version 2) epitope
ARTDLEMQI

SEQ ID NO: 108 - protein, 9 aa, Artificial Sequence
  Homo sapiens Keratin, type I cytoskeletal 17 (Cytokeratin 17) (K17) (CK 17) (Version 2) epitope
ASYLDKVRA

SEQ ID NO: 109 - protein, 9 aa, Artificial Sequence
  Homo sapiens Keratin, type I cytoskeletal 17 (Cytokeratin 17) (K17) (CK 17) (Version 2) epitope
DVNGLRRVL

SEQ ID NO: 110 - protein, 9 aa, Artificial Sequence
  Homo sapiens Keratin, type I cytoskeletal 17 (Cytokeratin 17) (K17) (CK 17) (Version 2) epitope
GLRRVLDEL

SEQ ID NO: 111 - protein, 12 aa, Artificial Sequence
  Homo sapiens Keratin, type I cytoskeletal 17 (Cytokeratin 17) (K17) (CK 17) (Version 2) epitope
ISSVLAGASCPA

SEQ ID NO: 112 - protein, 9 aa, Artificial Sequence
  Homo sapiens Keratin, type I cytoskeletal 17 (Cytokeratin 17) (K17) (CK 17) (Version 2) epitope
LDKVRALEE

SEQ ID NO: 113 - protein, 9 aa, Artificial Sequence
  Homo sapiens Keratin, type I cytoskeletal 17 (Cytokeratin 17) (K17) (CK 17) (Version 2) epitope
QIEGLKEEL

SEQ ID NO: 114 - protein, 12 aa, Artificial Sequence
  Homo sapiens Keratin, type I cytoskeletal 17 (Cytokeratin 17) (K17) (CK 17) (Version 2) epitope
RALEEANADLEV

SEQ ID NO: 115 - protein, 9 aa, Artificial Sequence
  Homo sapiens Keratin, type I cytoskeletal 17 (Cytokeratin 17) (K17) (CK 17) (Version 2) epitope
RLASYLDKV

SEQ ID NO: 116 - protein, 8 aa, Artificial Sequence
  Homo sapiens Keratin, type I cytoskeletal 17 (Cytokeratin 17) (K17) (CK 17) (Version 2) epitope
SYLDKVRA

SEQ ID NO: 117 - protein, 20 aa, Artificial Sequence
  Homo sapiens Keratin, type I cytoskeletal 17 (Cytokeratin 17) (K17) (CK 17) (Version 2) epitope
SYLDKVRALEEANADLEVKI

SEQ ID NO: 118 - protein, 9 aa, Artificial Sequence
  Homo sapiens maspin epitope
GLEKIEKQL

SEQ ID NO: 119 - protein, 10 aa, Artificial Sequence
  Homo sapiens maspin epitope
MGNIDSINCK

SEQ ID NO: 120 - protein, 9 aa, Artificial Sequence
  Homo sapiens maspin epitope
YSLKLIKRL

SEQ ID NO: 121 - protein, 20 aa, Artificial Sequence
  Homo sapiens MBP protein epitope
ASQKRPSQRHGSKYLATAST

SEQ ID NO: 122 - protein, 15 aa, Artificial Sequence
  Homo sapiens MBP protein epitope
ENPVVHFFKNIVTPR

SEQ ID NO: 123 - protein, 9 aa, Artificial Sequence
  Homo sapiens MBP protein epitope
VVHFFKNIV

SEQ ID NO: 124 - protein, 19 aa, Artificial Sequence
  Homo sapiens MBP protein epitope
DENPVVHFFKNIVTPRTPP

SEQ ID NO: 125 - protein, 20 aa, Artificial Sequence
  Homo sapiens MBP protein epitope
HHPARTAHYGSLPQKSHGRT

SEQ ID NO: 126 - protein, 20 aa, Artificial Sequence
  Homo sapiens MBP protein epitope
VVHFFKNIVTPRTPPPSQGK

SEQ ID NO: 127 - protein, 21 aa, Artificial Sequence
  Homo sapiens MBP protein epitope
ASQKRPSQRHGSKYLATASTM

SEQ ID NO: 128 - protein, 20 aa, Artificial Sequence
  Homo sapiens MBP protein epitope
FKGVDAQGTLSKIFKLGGRD

SEQ ID NO: 129 - protein, 19 aa, Artificial Sequence
  Homo sapiens MBP protein epitope
RPGFGYGGRASDYKSAHKG

SEQ ID NO: 130 - protein, 38 aa, Artificial Sequence
  Homo sapiens MBP protein epitope
ASQKRPSQRHGSKYLATASTMDHARHGFLPRHRDTGIL

SEQ ID NO: 131 - protein, 9 aa, Artificial Sequence
  Homo sapiens MBP protein epitope
KYLATASTM

SEQ ID NO: 132 - protein, 20 aa, Artificial Sequence
  Homo sapiens MBP protein epitope
GLSLSRFSWGAEGQRPGFGY

SEQ ID NO: 133 - protein, 43 aa, Artificial Sequence
  Homo sapiens MBP protein epitope
FGGDRGAPKRGSGKDSHHPARTAHYGSLPQKSHGRTQDENPVV

SEQ ID NO: 134 - protein, 40 aa, Artificial Sequence
  Homo sapiens MBP protein epitope
GLSLSRFSWGAEGQRPGFGYGGRASDYKSAHKGFKGVDAQ

SEQ ID NO: 135 - protein, 9 aa, Artificial Sequence
  Homo sapiens MHC class I related protein A epitope
AAAAAIFVI

SEQ ID NO: 136 - protein, 9 aa, Artificial Sequence
  Homo sapiens Myelin basic protein epitope
SLSRFSWGA

SEQ ID NO: 137 - protein, 9 aa, Artificial Sequence
  Homo sapiens Myelin basic protein epitope
DYKSAHKGF

SEQ ID NO: 138 - protein, 19 aa, Artificial Sequence
  Homo sapiens myelin basic protein epitope
SKIFKLGGRDSRSGSPMAR

SEQ ID NO: 139 - protein, 8 aa, Artificial Sequence
  Homo sapiens myelin basic protein epitope
TPRTPPPQ

SEQ ID NO: 140 - protein, 9 aa, Artificial Sequence
  Homo sapiens myelin proteolipid protein epitope
FLYGALLLA

SEQ ID NO: 141 - protein, 9 aa, Artificial Sequence
  Homo sapiens myelin proteolipid protein epitope
KLIETYFSK

SEQ ID NO: 142 - protein, 9 aa, Artificial Sequence
  Homo sapiens Myelin-associated glycoprotein precursor epitope
LMWAKIGPV

SEQ ID NO: 143 - protein, 9 aa, Artificial Sequence
  Homo sapiens Myelin-associated glycoprotein precursor epitope
SLLLELEEV

SEQ ID NO: 144 - protein, 9 aa, Artificial Sequence
  Homo sapiens Myelin-associated glycoprotein precursor epitope
VLFSSDFRI

SEQ ID NO: 145 - protein, 9 aa, Artificial Sequence
  Homo sapiens Myosin heavy chain, skeletal muscle, adult 2 (Myosin heavy chain IIa) (MyHC-IIa) epitope
EFQKMRRDL

SEQ ID NO: 146 - protein, 9 aa, Artificial Sequence
  Homo sapiens Myosin heavy chain, skeletal muscle, adult 2 (Myosin heavy chain IIa) (MyHC-IIa) epitope
KMRRDLEEA

SEQ ID NO: 147 - protein, 12 aa, Artificial Sequence
  Homo sapiens peroxiredoxin-2 isoform a epitope
EVKLSDYKGKYV

SEQ ID NO: 148 - protein, 10 aa, Artificial Sequence
  Homo sapiens proinsulin precursor epitope
HLCGSHLVEA

SEQ ID NO: 149 - protein, 10 aa, Artificial Sequence
  Homo sapiens proinsulin precursor epitope
ALWGPDPAAA

SEQ ID NO: 150 - protein, 9 aa, Artificial Sequence
  Homo sapiens proinsulin precursor epitope
RLLPLLALL

SEQ ID NO: 151 - protein, 10 aa, Artificial Sequence
  Homo sapiens proinsulin precursor epitope
ALWMRLLPLL

SEQ ID NO: 152 - protein, 10 aa, Artificial Sequence
  Homo sapiens proinsulin precursor epitope
WMRLLPLLAL

SEQ ID NO: 153 - protein, 10 aa, Artificial Sequence
  Homo sapiens proinsulin precursor epitope
PLALEGSLQK

SEQ ID NO: 154 - protein, 10 aa, Artificial Sequence
  Homo sapiens proinsulin precursor epitope
PLLALLALWG

SEQ ID NO: 155 - protein, 9 aa, Artificial Sequence
  Homo sapiens Receptor-type tyrosine-protein phosphatase-like N precursor epitope
LLPPLLEHL

SEQ ID NO: 156 - protein, 9 aa, Artificial Sequence
  Homo sapiens Receptor-type tyrosine-protein phosphatase-like N precursor epitope
SLAAGVKLL

SEQ ID NO: 157 - protein, 9 aa, Artificial Sequence
  Homo sapiens Receptor-type tyrosine-protein phosphatase-like N precursor epitope
SLSPLQAEL

SEQ ID NO: 158 - protein, 9 aa, Artificial Sequence
  Homo sapiens Receptor-type tyrosine-protein phosphatase-like N precursor epitope
ALTAVAEEV

SEQ ID NO: 159 - protein, 10 aa, Artificial Sequence
  Homo sapiens Receptor-type tyrosine-protein phosphatase-like N precursor epitope
SLYHVYEVNL

SEQ ID NO: 160 - protein, 9 aa, Artificial Sequence
  Homo sapiens Receptor-type tyrosine-protein phosphatase-like N precursor epitope
TIADFWQMV

SEQ ID NO: 161 - protein, 9 aa, Artificial Sequence
  Homo sapiens Receptor-type tyrosine-protein phosphatase-like N precursor epitope
VIVMLTPLV

SEQ ID NO: 162 - protein, 9 aa, Artificial Sequence
  Homo sapiens Receptor-type tyrosine-protein phosphatase-like N precursor epitope
MVWESGCTV

SEQ ID NO: 163 - protein, 14 aa, Artificial Sequence
  Homo sapiens S-arrestin epitope
FLGELTSSEVATEV

SEQ ID NO: 164 - protein, 20 aa, Artificial Sequence
  Homo sapiens S-arrestin epitope
FMSDKPLHLAVSLNKEIYFH

SEQ ID NO: 165 - protein, 15 aa, Artificial Sequence
  Homo sapiens S-arrestin epitope
GEAEEGKRDKNDVDE

SEQ ID NO: 166 - protein, 20 aa, Artificial Sequence
  Homo sapiens S-arrestin epitope
GEPIPVTVTVTNNTEKTVKK

SEQ ID NO: 167 - protein, 20 aa, Artificial Sequence
  Homo sapiens S-arrestin epitope
HPQPEDPAKESYQDANLVFE

SEQ ID NO: 168 - protein, 20 aa, Artificial Sequence
  Homo sapiens S-arrestin epitope
IKAFVEQVANVVLYSSDYYV

SEQ ID NO: 169 - protein, 20 aa, Artificial Sequence
  Homo sapiens S-arrestin epitope
KSSVRLLIRKVQHAPLEMGP

SEQ ID NO: 170 - protein, 20 aa, Artificial Sequence
  Homo sapiens S-arrestin epitope
QPRAEAAWQFFMSDKPLHLA

SEQ ID NO: 171 - protein, 20 aa, Artificial Sequence
  Homo sapiens S-arrestin epitope
SYQDANLVFEEFARHNLKDA

SEQ ID NO: 172 - protein, 20 aa, Artificial Sequence
  Homo sapiens S-arrestin epitope
TDAEEDKIPKKSSVRLLIRK

SEQ ID NO: 173 - protein, 20 aa, Artificial Sequence
  Homo sapiens S-arrestin epitope
TNNTEKTVKKIKAFVEQVAN

SEQ ID NO: 174 - protein, 20 aa, Artificial Sequence
  Homo sapiens S-arrestin epitope
VQHAPLEMGPQPRAEAAWQF

SEQ ID NO: 175 - protein, 20 aa, Artificial Sequence
  Homo sapiens S-arrestin epitope
VSLNKEIYFHGEPIPVTVTV

SEQ ID NO: 176 - protein, 20 aa, Artificial Sequence
  Homo sapiens S-arrestin epitope
VYVTLTCAFRYGQEDIDVIG

SEQ ID NO: 177 - protein, 20 aa, Artificial Sequence
  Homo sapiens S-arrestin epitope
YGQEDIDVIGLTFRRDLYFS

SEQ ID NO: 178 - protein, 10 aa, Artificial Sequence
  Homo sapiens SSA protein SS-56 epitope
YTCPLCRAPV

SEQ ID NO: 179 - protein, 8 aa, Artificial Sequence
  Homo sapiens Steroid 21-hydroxylase epitope
EPLARLEL

SEQ ID NO: 180 - protein, 20 aa, Artificial Sequence
  Homo sapiens Steroid 21-hydroxylase epitope
EPLARLELFVVLTRLLQAFT

SEQ ID NO: 181 - protein, 20 aa, Artificial Sequence
  Homo sapiens Steroid 21-hydroxylase epitope
IKDDNLMPAYYKCIQEVLKT

SEQ ID NO: 182 - protein, 20 aa, Artificial Sequence
  Homo sapiens Steroid 21-hydroxylase epitope
IRDSMEPVVEQLTQEFCERM

SEQ ID NO: 183 - protein, 8 aa, Artificial Sequence
  Homo sapiens T-cell receptor V beta chain 13.1 epitope
LGRAGLTY

SEQ ID NO: 184 - protein, 9 aa, Artificial Sequence
  Homo sapiens transaldolase 1 epitope
LLFSFAQAV

SEQ ID NO: 185 - protein, 9 aa, Artificial Sequence
  Homo sapiens Vasoactive intestinal polypeptide receptor 1 precursor epitope
RRKWRRWHL

SEQ ID NO: 186 - protein, 9 aa, Artificial Sequence
  Homo sapiens Vasoactive intestinal polypeptide receptor 1 precursor epitope
RRKWRRWHL

SEQ ID NO: 187 - protein, 20 aa, Artificial Sequence
  Arachis hypogaea 2S protein 1 epitope
AHASARQQWELQGDRRCQSQ

SEQ ID NO: 188 - protein, 20 aa, Artificial Sequence
  Arachis hypogaea 2S protein 1 epitope
AKLTILVALALFLLAAHASA

SEQ ID NO: 189 - protein, 19 aa, Artificial Sequence
  Arachis hypogaea 2S protein 1 epitope
ALQQIMENQSDRLQGRQQE

SEQ ID NO: 190 - protein, 20 aa, Artificial Sequence
  Arachis hypogaea 2S protein 1 epitope
ANLRPCEQHLMQKIQRDEDS

SEQ ID NO: 191 - protein, 20 aa, Artificial Sequence
  Arachis hypogaea 2S protein 1 epitope
CNELNEFENNQRCMCEALQQ

SEQ ID NO: 192 - protein, 16 aa, Artificial Sequence
  Homo sapiens 5-hydroxytryptamine receptor 2C (5-HT-2C) (Serotonin receptor 2C) (5-HT2C) (5-HTR2C) (5HT-1C) epitope
PRGTMQAINNERKASK

SEQ ID NO: 193 - protein, 12 aa, Artificial Sequence
  Bos taurus Allergen Bos d 2 precursor epitope
DQGTCLLLTEVA

SEQ ID NO: 194 - protein, 14 aa, Artificial Sequence
  Bos taurus Allergen Bos d 2 precursor epitope
ELEKYQQLNSERGV

SEQ ID NO: 195 - protein, 13 aa, Artificial Sequence
  Bos taurus Allergen Bos d 2 precursor epitope
GERITKMTEGLAK

SEQ ID NO: 196 - protein, 14 aa, Artificial Sequence
  Bos taurus Allergen Bos d 2 precursor epitope
PGEWRIIYAAADNK

SEQ ID NO: 197 - protein, 8 aa, Artificial Sequence
  Bos taurus Allergen Bos d 2 precursor epitope
RIECINDC

SEQ ID NO: 198 - protein, 12 aa, Artificial Sequence
  Bos taurus Allergen Bos d 2 precursor epitope
VAKRQEGYVYVL

SEQ ID NO: 199 - protein, 10 aa, Artificial Sequence
  Bos taurus Allergen Bos d 2 precursor epitope
VSENMLVTYV

SEQ ID NO: 200 - protein, 12 aa, Artificial Sequence
  Bos taurus Allergen Bos d 2 precursor epitope
DQGTCLLLTEVA

SEQ ID NO: 201 - protein, 14 aa, Artificial Sequence
  Bos taurus Allergen Bos d 2 precursor epitope
ELEKYQQLNSERGV

SEQ ID NO: 202 - protein, 16 aa, Artificial Sequence
  Bos taurus Allergen Bos d 2 precursor epitope
ELEKYQQLNSERGVPN

SEQ ID NO: 203 - protein, 13 aa, Artificial Sequence
  Bos taurus Allergen Bos d 2 precursor epitope
GERITKMTEGLAK

SEQ ID NO: 204 - protein, 14 aa, Artificial Sequence
  Bos taurus Allergen Bos d 2 precursor epitope
PGEWRIIYAAADNK

SEQ ID NO: 205 - protein, 8 aa, Artificial Sequence
  Bos taurus Allergen Bos d 2 precursor epitope
RIECINDC

SEQ ID NO: 206 - protein, 12 aa, Artificial Sequence
  Bos taurus Allergen Bos d 2 precursor epitope
VAKRQEGYVYVL

SEQ ID NO: 207 - protein, 10 aa, Artificial Sequence
  Bos taurus Allergen Bos d 2 precursor epitope
VSENMLVTYV

SEQ ID NO: 208 - protein, 13 aa, Artificial Sequence
  Cryptomeria japonica Allergen Cry j 2 epitope
DIFASKNFHLQKN

SEQ ID NO: 209 - protein, 13 aa, Artificial Sequence
  Cryptomeria japonica Allergen Cry j 2 epitope
GIIAAYQNPASWK

SEQ ID NO: 210 - protein, 12 aa, Artificial Sequence
  Cryptomeria japonica Allergen Cry j 2 epitope
KLTSGKIASCLN

SEQ ID NO: 211 - protein, 12 aa, Artificial Sequence
  Cryptomeria japonica Allergen Cry j 2 epitope
QFAKLTGFTLMG

SEQ ID NO: 212 - protein, 8 aa, Artificial Sequence
  Aspergillus fumigatus allergen I/a; Asp f I/a epitope
INQQLNPK

SEQ ID NO: 213 - protein, 15 aa, Artificial Sequence
  Aspergillus fumigatus allergen I/a; Asp f I/a epitope
INQQLNPKTNKWEDK

SEQ ID NO: 214 - protein, 11 aa, Artificial Sequence
  Aspergillus fumigatus allergen I/a; Asp f I/a epitope
LNPKTNKWEDK

SEQ ID NO: 215 - protein, 8 aa, Artificial Sequence
  Aspergillus fumigatus allergen I/a; Asp f I/a epitope
INQQLNPK

SEQ ID NO: 216 - protein, 15 aa, Artificial Sequence
  Aspergillus fumigatus allergen I/a; Asp f I/a epitope
INQQLNPKTNKWEDK

SEQ ID NO: 217 - protein, 11 aa, Artificial Sequence
  Aspergillus fumigatus allergen I/a; Asp f I/a epitope
LNPKTNKWEDK

SEQ ID NO: 218 - protein, 7 aa, Artificial Sequence
  Aspergillus fumigatus allergen I/a; Asp f I/a epitope
TNKWEDK

SEQ ID NO: 219 - protein, 12 aa, Artificial Sequence
  Aspergillus fumigatus allergen I/a; Asp f I/a epitope
LNPKTNKWEDKR

SEQ ID NO: 220 - protein, 15 aa, Artificial Sequence
  Dermatophagoides farinae Allergen Mag epitope
PRLSWHQYTKRDSRE

SEQ ID NO: 221 - protein, 15 aa, Artificial Sequence
  Dermatophagoides farinae Allergen Mag epitope
TVDLISPVTKRASLK

SEQ ID NO: 222 - protein, 18 aa, Artificial Sequence
  Bos taurus Alpha-S1-casein precursor epitope
AWYYVPLGTQYTDAPSFS

SEQ ID NO: 223 - protein, 18 aa, Artificial Sequence
  Bos taurus Alpha-S1-casein precursor epitope
DAYPSGAWYYVPLGTQYT

SEQ ID NO: 224 - protein, 18 aa, Artificial Sequence
  Bos taurus Alpha-S1-casein precursor epitope
DIGSESTEDQAMEDIKQM

SEQ ID NO: 225 - protein, 6 aa, Artificial Sequence
  Bos taurus Alpha-S1-casein precursor epitope
EDIKQM

SEQ ID NO: 226 - protein, 12 aa, Artificial Sequence
  Bos taurus Alpha-S1-casein precursor epitope
EPMIGVNQELAY

SEQ ID NO: 227 - protein, 18 aa, Artificial Sequence
  Bos taurus Alpha-S1-casein precursor epitope
EPMIGVNQELAYFYPELF

SEQ ID NO: 228 - protein, 17 aa, Artificial Sequence
  Arachis hypogaea Ara h 2.01 allergen epitope
ELNEFENNQRCMCEALQ

SEQ ID NO: 229 - protein, 16 aa, Artificial Sequence
  Arachis hypogaea Ara h 2.01 allergen epitope
SQLERANLRPCEQHLM

SEQ ID NO: 230 - protein, 15 aa, Artificial Sequence
  Cryptomeria japonica Cry j 1 precursor epitope
GATRDRPLWIIFSGN

SEQ ID NO: 231 - protein, 20 aa, Artificial Sequence
  Cryptomeria japonica Cry j 1 precursor epitope
IFSGNMNIKLKMPMYIAGYK

SEQ ID NO: 232 - protein, 20 aa, Artificial Sequence
  Cryptomeria japonica Cry j 1 precursor epitope
KMPMYIAGYKTFDGRGAQVY

SEQ ID NO: 233 - protein, 20 aa, Artificial Sequence
  Cryptomeria japonica Cry j 1 precursor epitope
LGHDDAYSDDKSMKVTVAFN

SEQ ID NO: 234 - protein, 19 aa, Artificial Sequence
  Cryptomeria japonica Cry j 1 precursor epitope
SGKYEGGNIYTKKEAFNVE

SEQ ID NO: 235 - protein, 11 aa, Artificial Sequence
  Cochliobolus lunatus Cytochrome c epitope
ENPKKYIPGTK

SEQ ID NO: 236 - protein, 11 aa, Artificial Sequence
  Cochliobolus lunatus Cytochrome c epitope
GLFGRKTGSVA

SEQ ID NO: 237 - protein, 9 aa, Artificial Sequence
  Cochliobolus lunatus Cytochrome c epitope
KIGPELHGL

SEQ ID NO: 238 - protein, 12 aa, Artificial Sequence
  Cochliobolus lunatus Cytochrome c epitope
LKAGEGNKIGPE

SEQ ID NO: 239 - protein, 11 aa, Artificial Sequence
  Cochliobolus lunatus Cytochrome c epitope
LKKPKDRNDLI

SEQ ID NO: 240 - protein, 18 aa, Artificial Sequence
  Dermatophagoides farinae Der f 2 allergen epitope
GLEIDVPGIDTNACHFVK

SEQ ID NO: 241 - protein, 20 aa, Artificial Sequence
  Dermatophagoides farinae Der f 2 allergen epitope
PGIDTNACHFVKCPLVKGQQ

SEQ ID NO: 242 - protein, 19 aa, Artificial Sequence
  Dermatophagoides pteronyssinus Der p 1 allergen epitope
RFGISNYCQIYPPNANKIR

SEQ ID NO: 243 - protein, 15 aa, Artificial Sequence
  Dermatophagoides pteronyssinus Der p 1 allergen epitope
AVNIVGYSNAQGVDY

SEQ ID NO: 244 - protein, 20 aa, Artificial Sequence
  Chironomus thummi globin Ctt 3-1 epitope
FAGKDLESIKGTAPFETHAN

SEQ ID NO: 245 - protein, 11 aa, Artificial Sequence
  Chironomus thummi globin Ctt 3-1 epitope
GTAPFETHANR

SEQ ID NO: 246 - protein, 21 aa, Artificial Sequence
  Chironomus thummi globin Ctt 3-1 epitope
KGTAPFETHANRIVGFFSKII

SEQ ID NO: 247 - protein, 21 aa, Artificial Sequence
  Chironomus thummi thummi Globin CTT-III epitope
AHTDFAGAEAAWGATLDTFFG

SEQ ID NO: 248 - protein, 20 aa, Artificial Sequence
  Chironomus thummi thummi Globin CTT-III epitope
FAGKDLESIKGTAPFEIHAN

SEQ ID NO: 249 - protein, 21 aa, Artificial Sequence
  Chironomus thummi thummi Globin CTT-III epitope
VNTFVASHKPRGVTHDQLNNF

SEQ ID NO: 250 - protein, 8 aa, Artificial Sequence
  Chironomus thummi thummi Globin CTT-III precursor epitope
ADPSIMAK

SEQ ID NO: 251 - protein, 21 aa, Artificial Sequence
  Chironomus thummi thummi Globin CTT-III precursor epitope
ADPSIMAKFTQFAGKDLESIK

SEQ ID NO: 252 - protein, 5 aa, Artificial Sequence
  Chironomus thummi thummi Globin CTT-III precursor epitope
AEAAW

SEQ ID NO: 253 - protein, 20 aa, Artificial Sequence
  Chironomus thummi thummi Globin CTT-III precursor epitope
AEAAWGATLDTFFGMIFSKM

SEQ ID NO: 254 - protein, 8 aa, Artificial Sequence
  Chironomus thummi thummi Globin CTT-III precursor epitope
AGFVSYMK

SEQ ID NO: 255 - protein, 15 aa, Artificial Sequence
  Phaseolus vulgaris Glycine-rich cell wall structural protein 1.8 precursor epitope
GGYGDGGAHGGGYGG

SEQ ID NO: 256 - protein, 15 aa, Artificial Sequence
  Phleum pratense Group V allergen Phl p 5 epitope
ATPEAKYDAYVATLS

SEQ ID NO: 257 - protein, 15 aa, Artificial Sequence
  Phleum pratense Group V allergen Phl p 5 epitope
FTVFEAAFNNAIKAG

SEQ ID NO: 258 - protein, 15 aa, Artificial Sequence
  Phleum pratense Group V allergen Phl p 5 epitope
KYDAYVATLSEALRI

SEQ ID NO: 259 - protein, 15 aa, Artificial Sequence
  Phleum pratense Group V allergen Phl p 5 epitope
PANDKFTVFEAAFNN

SEQ ID NO: 260 - protein, 15 aa, Artificial Sequence
  Phleum pratense Group V allergen Phl p 5 epitope
PKGGAESSSKAALTS

SEQ ID NO: 261 - protein, 16 aa, Artificial Sequence
  Homo sapiens KIAA1224 protein epitope
DLESYLQLNCERGTWR

SEQ ID NO: 262 - protein, 15 aa, Artificial Sequence
  Lepidoglyphus destructor Lep D 2 precursor epitope
KGEALDFNYGMTIPA

SEQ ID NO: 263 - protein, 12 aa, Artificial Sequence
  Corylus avellana lipid transfer protein precursor epitope
AGLPGKCGVNIP

SEQ ID NO: 264 - protein, 12 aa, Artificial Sequence
  Corylus avellana lipid transfer protein precursor epitope
AKGIAGLNPNLA

SEQ ID NO: 265 - protein, 12 aa, Artificial Sequence
  Corylus avellana lipid transfer protein precursor epitope
CGVNIPYKISPS

SEQ ID NO: 266 - protein, 12 aa, Artificial Sequence
  Corylus avellana lipid transfer protein precursor epitope
CKGVRAVNDASR

SEQ ID NO: 267 - protein, 12 aa, Artificial Sequence
  Corylus avellana lipid transfer protein precursor epitope
CVLYLKNGGVLP

SEQ ID NO: 268 - protein, 16 aa, Artificial Sequence
  Homo sapiens Lipocalin 1 (tear prealbumin) epitope
KPVRGVKLVGRDPKNN

SEQ ID NO: 269 - protein, 15 aa, Artificial Sequence
  Dermatophagoides farinae Mag3 epitope
EFNTEFTIHADKNNL

SEQ ID NO: 270 - protein, 15 aa, Artificial Sequence
  Dermatophagoides farinae Mag3 epitope
FTIHADKNNLKMHMD

SEQ ID NO: 271 - protein, 15 aa, Artificial Sequence
  Dermatophagoides farinae Mag3 epitope
KMHMDFPNVFQADLT

SEQ ID NO: 272 - protein, 13 aa, Artificial Sequence
  Apium graveolens Major allergen Api g 1 epitope
ALFKALEAYLIAN

SEQ ID NO: 273 - protein, 12 aa, Artificial Sequence
  Apium graveolens Major allergen Api g 1 epitope
DAVVPEENIKYA

SEQ ID NO: 274 - protein, 12 aa, Artificial Sequence
  Apium graveolens Major allergen Api g 1 epitope
DILLGFIESIEN

SEQ ID NO: 275 - protein, 12 aa, Artificial Sequence
  Apium graveolens Major allergen Api g 1 epitope
GGSICKTTAIFH

SEQ ID NO: 276 - protein, 12 aa, Artificial Sequence
  Apium graveolens Major allergen Api g 1 epitope
GVQTHVLELTSS

SEQ ID NO: 277 - protein, 15 aa, Artificial Sequence
  Aspergillus fumigatus Major allergen Asp f 2 precursor epitope
FGNRPTMEAVGAYDV

SEQ ID NO: 278 - protein, 15 aa, Artificial Sequence
  Aspergillus fumigatus Major allergen Asp f 2 precursor epitope
MEAVGAYDVIVNGDK

SEQ ID NO: 279 - protein, 16 aa, Artificial Sequence
  Canis lupus familiaris Major allergen Can f 1 precursor epitope
ALEDFREFSRAKGLNQ

SEQ ID NO: 280 - protein, 16 aa, Artificial Sequence
  Canis lupus familiaris Major allergen Can f 1 precursor epitope
DQEVPEKPDSVTPMIL

SEQ ID NO: 281 - protein, 12 aa, Artificial Sequence
  Corylus avellana major allergen Cor a 1.0401 epitope
AGKEKAAGLFKA

SEQ ID NO: 282 - protein, 12 aa, Artificial Sequence
  Corylus avellana major allergen Cor a 1.0401 epitope
AGLFKAVEAYLL

SEQ ID NO: 283 - protein, 12 aa, Artificial Sequence
  Corylus avellana major allergen Cor a 1.0401 epitope
APQHFTSAENLE

SEQ ID NO: 284 - protein, 12 aa, Artificial Sequence
  Corylus avellana major allergen Cor a 1.0401 epitope
ARLFKSFVLDAD

SEQ ID NO: 285 - protein, 12 aa, Artificial Sequence
  Corylus avellana major allergen Cor a 1.0401 epitope
EIDHANFKYCYS

SEQ ID NO: 286 - protein, 13 aa, Artificial Sequence
  Daucus carota Major allergen Dau c 1 epitope
ALFKAIEAYLIAN

SEQ ID NO: 287 - protein, 16 aa, Artificial Sequence
  Equus caballus Major allergen Equ c 1 precursor epitope
DGYNVFRISEFENDEH

SEQ ID NO: 288 - protein, 16 aa, Artificial Sequence
  Equus caballus Major allergen Equ c 1 precursor epitope
DKDRPFQLFEFYAREP

SEQ ID NO: 289 - protein, 16 aa, Artificial Sequence
  Equus caballus Major allergen Equ c 1 precursor epitope
DLTKIDRCFQLRGNGV

SEQ ID NO: 290 - protein, 16 aa, Artificial Sequence
  Equus caballus Major allergen Equ c 1 precursor epitope
DRPFQLFEFYAREPDV

SEQ ID NO: 291 - protein, 16 aa, Artificial Sequence
  Equus caballus Major allergen Equ c 1 precursor epitope
DVSPEIKEEFVKIVQK

SEQ ID NO: 292 - protein, 17 aa, Artificial Sequence
  Felis catus major allergen I epitope
ENARILKNCVDAKMTEE

SEQ ID NO: 293 - protein, 17 aa, Artificial Sequence
  Felis catus major allergen I epitope
RDVDLFLTGTPDEYVEQ

SEQ ID NO: 294 - protein, 17 aa, Artificial Sequence
  Felis catus major allergen I epitope
TGTPDEYVEQVAQYKAL

SEQ ID NO: 295 - protein, 17 aa, Artificial Sequence
  Felis catus Major allergen I polypeptide chain 1 precursor epitope
DVDLFLTGTPDEYVEQV

SEQ ID NO: 296 - protein, 17 aa, Artificial Sequence
  Felis catus Major allergen I polypeptide chain 1 precursor epitope
EICPAVKRDVDLFLTGT

SEQ ID NO: 297 - protein, 16 aa, Artificial Sequence
  Felis catus Major allergen I polypeptide chain 1 precursor epitope
EQVAQYKALPVVLENA

SEQ ID NO: 298 - protein, 17 aa, Artificial Sequence
  Felis catus Major allergen I polypeptide chain 1 precursor epitope
KALPVVLENARILKNCV

SEQ ID NO: 299 - protein, 17 aa, Artificial Sequence
  Felis catus Major allergen I polypeptide chain 1 precursor epitope
LFLTGTPDEYVEQVAQY

SEQ ID NO: 300 - protein, 16 aa, Artificial Sequence
  Felis catus major allergen I, polypeptide chain 1 epitope
KENALSLLDKIYTSPL

SEQ ID NO: 301 - protein, 16 aa, Artificial Sequence
  Felis catus major allergen I, polypeptide chain 1 epitope
KMTEEDKENALSLLDK

SEQ ID NO: 302 - protein, 15 aa, Artificial Sequence
  Malus x domestica Major allergen Mal d 1 epitope
GLFKLIESYLKDHPD

SEQ ID NO: 303 - protein, 15 aa, Artificial Sequence
  Prunus avium Major allergen Pru av 1 epitope
NLFKLIETYLKGHPD

SEQ ID NO: 304 - protein, 20 aa, Artificial Sequence
  Hevea brasiliensis Major latex allergen Hev b 5 epitope
AAPAEGEKPAEEEKPITEAA

SEQ ID NO: 305 - protein, 20 aa, Artificial Sequence
  Hevea brasiliensis Major latex allergen Hev b 5 epitope
AEEEKPITEAAETATTEVPV

SEQ ID NO: 306 - protein, 20 aa, Artificial Sequence
  Hevea brasiliensis Major latex allergen Hev b 5 epitope
APAEPEAPAPETEKAEEVEK

SEQ ID NO: 307 - protein, 20 aa, Artificial Sequence
  Hevea brasiliensis Major latex allergen Hev b 5 epitope
APEADQTTPEEKPAEPEPVA

SEQ ID NO: 308 - protein, 20 aa, Artificial Sequence
  Hevea brasiliensis Major latex allergen Hev b 5 epitope
ASEQETADATPEKEEPTAAP

SEQ ID NO: 309 - protein, 11 aa, Artificial Sequence
  Dermatophagoides pteronyssinus Major mite fecal allergen Der p 1 epitope
YAYVAREQSCR

SEQ ID NO: 310 - protein, 19 aa, Artificial Sequence
  Dermatophagoides pteronyssinus Major mite fecal allergen Der p 1 epitope
ALAQTHTAIAVIIGIKDLD

SEQ ID NO: 311 - protein, 35 aa, Artificial Sequence
  Olea europaea Major pollen allergen epitope
EDIPQPPVSQFHIQGQVYCDTCRAGFITELSEFIP

SEQ ID NO: 312 - protein, 31 aa, Artificial Sequence
  Olea europaea Major pollen allergen epitope
GASLRLQCKDKENGDVTFTEVGYTRAEGLYS

SEQ ID NO: 313 - protein, 34 aa, Artificial Sequence
  Olea europaea Major pollen allergen epitope
GTTRTVNPLGFFKKEALPKCAQVYNKLGMYPPNM

SEQ ID NO: 314 - protein, 53 aa, Artificial Sequence
  Olea europaea Major pollen allergen epitope
LVERDHKNEFCEITLISSGRKDCNEIPTEGWAKPSLKFKLNTVNGTTRTVNPL

SEQ ID NO: 315 - protein, 33 aa, Artificial Sequence
  Olea europaea Major pollen allergen epitope
MLVERDHKNEFCEITLISSGRKDCNEIPTEGWA

SEQ ID NO: 316 - protein, 12 aa, Artificial Sequence
  Artemisia vulgaris Major pollen allergen Art v 1 precursor epitope
AGGSPSPPADGG

SEQ ID NO: 317 - protein, 12 aa, Artificial Sequence
  Artemisia vulgaris Major pollen allergen Art v 1 precursor epitope
AGSKLCEKTSKT

SEQ ID NO: 318 - protein, 12 aa, Artificial Sequence
  Artemisia vulgaris Major pollen allergen Art v 1 precursor epitope
CDKKCIEWEKAQ

SEQ ID NO: 319 - protein, 12 aa, Artificial Sequence
  Artemisia vulgaris Major pollen allergen Art v 1 precursor epitope
DGGSPPPPADGG

SEQ ID NO: 320 - protein, 12 aa, Artificial Sequence
  Artemisia vulgaris Major pollen allergen Art v 1 precursor epitope
EKTSKTYSGKCD

SEQ ID NO: 321 - protein, 12 aa, Artificial Sequence
  Betula pendula Major pollen allergen Bet v 1-A epitope
AARLFKAFILDG

SEQ ID NO: 322 - protein, 15 aa, Artificial Sequence
  Betula pendula Major pollen allergen Bet v 1-A epitope
AARLFKAFILDGDNL

SEQ ID NO: 323 - protein, 12 aa, Artificial Sequence
  Betula pendula Major pollen allergen Bet v 1-A epitope
AEQVKASKEMGE

SEQ ID NO: 324 - protein, 21 aa, Artificial Sequence
  Betula pendula Major pollen allergen Bet v 1-A epitope
AFILDGDNLFPKVAPQAISSV

SEQ ID NO: 325 - protein, 12 aa, Artificial Sequence
  Betula pendula Major pollen allergen Bet v 1-A epitope
AISSVENIEGNG

SEQ ID NO: 326 - protein, 15 aa, Artificial Sequence
  Betula pendula Major pollen allergen Bet v 1-A epitope
ETLLRAVESYLLAHS

SEQ ID NO: 327 - protein, 16 aa, Artificial Sequence
  Betula pendula Major pollen allergen Bet v 1-F/I epitope
GETLLRAVESYLLAHS

SEQ ID NO: 328 - protein, 20 aa, Artificial Sequence
  Chamaecyparis obtusa Major pollen allergen Cha o 1 precursor epitope
ANNNYDPWSIYAIGGSSNPT

SEQ ID NO: 329 - protein, 20 aa, Artificial Sequence
  Chamaecyparis obtusa Major pollen allergen Cha o 1 precursor epitope
ASTGVTISNNHFFNHHKVML

SEQ ID NO: 330 - protein, 20 aa, Artificial Sequence
  Chamaecyparis obtusa Major pollen allergen Cha o 1 precursor epitope
CANWVWRSTQDSFNNGAYFV

SEQ ID NO: 331 - protein, 20 aa, Artificial Sequence
  Chamaecyparis obtusa Major pollen allergen Cha o 1 precursor epitope
DAITMRNVTDVWIDHNSLSD

SEQ ID NO: 332 - protein, 20 aa, Artificial Sequence
  Chamaecyparis obtusa Major pollen allergen Cha o 1 precursor epitope
DANWDQNRMKLADCAVGFGS

SEQ ID NO: 333 - protein, 20 aa, Artificial Sequence
  Cynodon dactylon Major pollen allergen Cyn d 1 epitope
AIGDKPGPNITATYGNKWLE

SEQ ID NO: 334 - protein, 20 aa, Artificial Sequence
  Cynodon dactylon Major pollen allergen Cyn d 1 epitope
CYEIKCKEPVECSGEPVLVK

SEQ ID NO: 335 - protein, 20 aa, Artificial Sequence
  Cynodon dactylon Major pollen allergen Cyn d 1 epitope
DHGGACGYKDVDKPPFDGMT

SEQ ID NO: 336 - protein, 20 aa, Artificial Sequence
  Cynodon dactylon Major pollen allergen Cyn d 1 epitope
EGGAHLVQDDVIPANWKPDT

SEQ ID NO: 337 - protein, 20 aa, Artificial Sequence
  Cynodon dactylon Major pollen allergen Cyn d 1 epitope
FKDGLGCGACYEIKCKEPVE

SEQ ID NO: 338 - protein, 15 aa, Artificial Sequence
  Phleum pratense Major pollen allergen Phl p 4 precursor epitope
FAEYKSDYVYQPFPK

SEQ ID NO: 339 - protein, 15 aa, Artificial Sequence
  Phleum pratense Major pollen allergen Phl p 4 precursor epitope
MLLRKYGIAAENVID

SEQ ID NO: 340 - protein, 15 aa, Artificial Sequence
  Phleum pratense Major pollen allergen Phl p 4 precursor epitope
NSFKPFAEYKSDYVY

SEQ ID NO: 341 - protein, 20 aa, Artificial Sequence
  Rattus norvegicus Major urinary protein precursor epitope
ASNKREKIEENGSMRVFMQH

SEQ ID NO: 342 - protein, 20 aa, Artificial Sequence
  Rattus norvegicus Major urinary protein precursor epitope
DIKEKFAKLCEAHGITRDNI

SEQ ID NO: 343 - protein, 20 aa, Artificial Sequence
  Rattus norvegicus Major urinary protein precursor epitope
EEASSTRGNLDVAKLNGDWF

SEQ ID NO: 344 - protein, 20 aa, Artificial Sequence
  Rattus norvegicus Major urinary protein precursor epitope
EENGSMRVFMQHIDVLENSL

SEQ ID NO: 345 - protein, 20 aa, Artificial Sequence
  Rattus norvegicus Major urinary protein precursor epitope
ENSLGFKFRIKENGECRELY

SEQ ID NO: 346 - protein, 21 aa, Artificial Sequence
  Dermatophagoides farinae Mite group 2 allergen Der f 2 precursor epitope
DIKYTWNVPKIAPKSENVVVT

SEQ ID NO: 347 - protein, 17 aa, Artificial Sequence
  Dermatophagoides farinae Mite group 2 allergen Der f 2 precursor epitope
DNGVLACAIATHGKIRD

SEQ ID NO: 348 - protein, 21 aa, Artificial Sequence
  Dermatophagoides farinae Mite group 2 allergen Der f 2 precursor epitope
EALFDANQNTKTAKIEIKASL

SEQ ID NO: 349 - protein, 45 aa, Artificial Sequence
  Dermatophagoides farinae Mite group 2 allergen Der f 2 precursor epitope
QYDIKYTWNVPKIAPKSENVVVTVKLIGDNGVLACAIATHGKIRD

SEQ ID NO: 350 - protein, 19 aa, Artificial Sequence
  Dermatophagoides farinae Mite group 2 allergen Der f 2 precursor epitope
TKTAKIEIKASLDGLEIDV

SEQ ID NO: 351 - protein, 14 aa, Artificial Sequence
  Dermatophagoides pteronyssinus Mite group 2 allergen Der p 2 epitope
ASIDGLGVDVPGID

SEQ ID NO: 352 - protein, 15 aa, Artificial Sequence
  Dermatophagoides pteronyssinus Mite group 2 allergen Der p 2 epitope
FEAVQNTKTAKIEIK

SEQ ID NO: 353 - protein, 17 aa, Artificial Sequence
  Dermatophagoides pteronyssinus Mite group 2 allergen Der p 2 epitope
RGKPPQLEAVFEAVQNT

SEQ ID NO: 354 - protein, 15 aa, Artificial Sequence
  Dermatophagoides pteronyssinus Mite group 2 allergen Der p 2 precursor epitope
CHGSEPCIIHRGKPF

SEQ ID NO: 355 - protein, 27 aa, Artificial Sequence
  Dermatophagoides pteronyssinus Mite group 2 allergen Der p 2 precursor epitope
CPLVKGQQYDIKYTWNVPKIAPKSENV

SEQ ID NO: 356 - protein, 26 aa, Artificial Sequence
  Dermatophagoides pteronyssinus Mite group 2 allergen Der p 2 precursor epitope
DIKYTWNVPKIAPKSENVVVTVKVMG

SEQ ID NO: 357 - protein, 15 aa, Artificial Sequence
  Dermatophagoides pteronyssinus Mite group 2 allergen Der p 2 precursor epitope
DQVDVKDCANHEIKK

SEQ ID NO: 358 - protein, 20 aa, Artificial Sequence
  Dermatophagoides pteronyssinus Mite group 2 allergen Der p 2 precursor epitope
DQVDVKDCANHEIKKVLVPG

SEQ ID NO: 359 - protein, 15 aa, Artificial Sequence
  Dermatophagoides pteronyssinus Mite group 2 allergen Der p 2 precursor epitope
CHGSEPCIIHRGKPF

SEQ ID NO: 360 - protein, 15 aa, Artificial Sequence
  Lepidoglyphus destructor Mite group 2 allergen Lep d 2 precursor epitope
DHGVMACGTVHGQVE

SEQ ID NO: 361 - protein, 15 aa, Artificial Sequence
  Lepidoglyphus destructor Mite group 2 allergen Lep d 2 precursor epitope
GCKFIKCPVKKGEAL

SEQ ID NO: 362 - protein, 15 aa, Artificial Sequence
  Lepidoglyphus destructor Mite group 2 allergen Lep d 2 precursor epitope
GEKMTLEAKFAANQD

SEQ ID NO: 363 - protein, 15 aa, Artificial Sequence
  Lepidoglyphus destructor Mite group 2 allergen Lep d 2 precursor epitope
GEVTELDITGCSGDT

SEQ ID NO: 364 - protein, 15 aa, Artificial Sequence
  Lepidoglyphus destructor Mite group 2 allergen Lep d 2 precursor epitope
GKMTFKDCGHGEVTE

SEQ ID NO: 365 - protein, 16 aa, Artificial Sequence
  Homo sapiens Neurofilament heavy polypeptide (NF-H) (Neurofilament triplet H protein) (200 kDa neurofilament protein) epitope
YQEAIQQLDAELRNTK

SEQ ID NO: 366 - protein, 10 aa, Artificial Sequence
  Prunus persica Non-specific lipid-transfer protein 1 epitope
AAALPGKCGV

SEQ ID NO: 367 - protein, 10 aa, Artificial Sequence
  Prunus persica Non-specific lipid-transfer protein 1 epitope
ACCNGIRNVN

SEQ ID NO: 368 - protein, 10 aa, Artificial Sequence
  Prunus persica Non-specific lipid-transfer protein 1 epitope
APCIPYVRGG

SEQ ID NO: 369 - protein, 10 aa, Artificial Sequence
  Prunus persica Non-specific lipid-transfer protein 1 epitope
IRNVNNLART

SEQ ID NO: 370 - protein, 11 aa, Artificial Sequence
  Prunus persica Non-specific lipid-transfer protein 1 epitope
ISASTNCATVK

SEQ ID NO: 371 - protein, 10 aa, Artificial Sequence
  Prunus persica Non-specific lipid-transfer protein 1 epitope
NLARTTPDRQ

SEQ ID NO: 372 - protein, 10 aa, Artificial Sequence
  Gallus gallus Ovalbumin epitope
CFDVFKELKV

SEQ ID NO: 373 - protein, 10 aa, Artificial Sequence
  Gallus gallus Ovalbumin epitope
GSIGAASMEF

SEQ ID NO: 374 - protein, 18 aa, Artificial Sequence
  Gallus gallus Ovalbumin epitope
IGLFRVASMASEKMKILE

SEQ ID NO: 375 - protein, 18 aa, Artificial Sequence
  Gallus gallus Ovalbumin epitope
IKHIATNAVLFFGRCVSP

SEQ ID NO: 376 - protein, 13 aa, Artificial Sequence
  Gallus gallus Ovalbumin epitope
IMSALAMVYLGAK

SEQ ID NO: 377 - protein, 14 aa, Artificial Sequence
  Gallus gallus Ovomucoid precursor epitope
AEVDCSRFPNATDK

SEQ ID NO: 378 - protein, 14 aa, Artificial Sequence
  Gallus gallus Ovomucoid precursor epitope
ATDKEGKDVLVCNK

SEQ ID NO: 379 - protein, 17 aa, Artificial Sequence
  Gallus gallus Ovomucoid precursor epitope
AVVESNGTLTLSHFGKC

SEQ ID NO: 380 - protein, 16 aa, Artificial Sequence
  Gallus gallus Ovomucoid precursor epitope
CLLCAYSIEFGTNISK

SEQ ID NO: 381 - protein, 20 aa, Artificial Sequence
  Gallus gallus Ovomucoid precursor epitope
DNECLLCAHKVEQGASVDKR

SEQ ID NO: 382 - protein, 16 aa, Artificial Sequence
  Musa acuminata pectate lyase epitope
GHSDELTSDKSMQVTI

SEQ ID NO: 383 - protein, 16 aa, Artificial Sequence
  Zinnia violacea Pectate lyase precursor epitope
GHSDSYTQDKNMQVTI

SEQ ID NO: 384 - protein, 21 aa, Artificial Sequence
  Dermatophagoides farinae Peptidase 1 precursor (Major mite fecal allergen Der f 1) (Allergen Der f I) epitope
DGRTIIQHDNGYQPNYHAVNI

SEQ ID NO: 385 - protein, 19 aa, Artificial Sequence
  Dermatophagoides farinae Peptidase 1 precursor (Major mite fecal allergen Der f 1) (Allergen Der f I) epitope
DLRSLRTVTPIRMQGGCGS

SEQ ID NO: 386 - protein, 19 aa, Artificial Sequence
  Dermatophagoides farinae Peptidase 1 precursor (Major mite fecal allergen Der f 1) (Allergen Der f I) epitope
GCGSCWAFSGVAATESAYL

SEQ ID NO: 387 - protein, 21 aa, Artificial Sequence
  Dermatophagoides farinae Peptidase 1 precursor (Major mite fecal allergen Der f 1) (Allergen Der f I) epitope
IREALTQTHTAIAVIIGIKDL

SEQ ID NO: 388 - protein, 19 aa, Artificial Sequence
  Dermatophagoides farinae Peptidase 1 precursor (Major mite fecal allergen Der f 1) (Allergen Der f I) epitope
IRMQGGCGSCWAFSGVAAT

SEQ ID NO: 389 - protein, 19 aa, Artificial Sequence
  Euroglyphus maynei Peptidase 1 precursor (Mite group 1 allergen Eur m 1) (Allergen Eur m I) epitope
FRHYDGRTIMQHDNGYQPN

SEQ ID NO: 390 - protein, 19 aa, Artificial Sequence
  Euroglyphus maynei Peptidase 1 precursor (Mite group 1 allergen Eur m 1) (Allergen Eur m I) epitope
GRTIMQHDNGYQPNYHAVN

SEQ ID NO: 391 - protein, 19 aa, Artificial Sequence
  Euroglyphus maynei Peptidase 1 precursor (Mite group 1 allergen Eur m 1) (Allergen Eur m I) epitope
HAVNIVGYGNTQGVDYWIV

SEQ ID NO: 392 - protein, 19 aa, Artificial Sequence
  Euroglyphus maynei Peptidase 1 precursor (Mite group 1 allergen Eur m 1) (Allergen Eur m I) epitope
NKIRQALTQTHTAVAVIIG

SEQ ID NO: 393 - protein, 19 aa, Artificial Sequence
  Euroglyphus maynei Peptidase 1 precursor (Mite group 1 allergen Eur m 1) (Allergen Eur m I) epitope
PYVAREQSCHRPNAQRYGL

SEQ ID NO: 394 - protein, 15 aa, Artificial Sequence
  Phleum pratense Phl p 3 allergen epitope
AVQVTFTVQKGSDPK

SEQ ID NO: 395 - protein, 15 aa, Artificial Sequence
  Phleum pratense Phl p 3 allergen epitope
EEWEPLTKKGNVWEV

SEQ ID NO: 396 - protein, 15 aa, Artificial Sequence
  Phleum pratense Phl p 3 allergen epitope
FTVQKGSDPKKLVLD

SEQ ID NO: 397 - protein, 15 aa, Artificial Sequence
  Phleum pratense Phl p 3 allergen epitope
FTVQKGSDPKKLVLN

SEQ ID NO: 398 - protein, 15 aa, Artificial Sequence
  Phleum pratense Phl p 3 allergen epitope
GSDPKKLVLDIKYTR

SEQ ID NO: 399 - protein, 15 aa, Artificial Sequence
  Apis mellifera Phospholipase A2 precursor epitope
CDCDDKFYDCLKNSA

SEQ ID NO: 400 - protein, 12 aa, Artificial Sequence
  Apis mellifera Phospholipase A2 precursor epitope
CLHYTVDKSKPK

SEQ ID NO: 401 - protein, 15 aa, Artificial Sequence
  Apis mellifera Phospholipase A2 precursor epitope
CRTHDMCPDVMSAGE

SEQ ID NO: 402 - protein, 18 aa, Artificial Sequence
  Apis mellifera Phospholipase A2 precursor epitope
DTISSYFVGKMYFNLIDT

SEQ ID NO: 403 - protein, 18 aa, Artificial Sequence
  Apis mellifera Phospholipase A2 precursor epitope
ERTEGRCLHYTVDKSKPK

SEQ ID NO: 404 - protein, 16 aa, Artificial Sequence
  Spiroplasma citri plectrovirus spv1-r8a2b orf 14 transmembrane protein epitope
HVIEVQQINSERSWFF

SEQ ID NO: 405 - protein, 20 aa, Artificial Sequence
  Lolium perenne pollen allergen epitope
CGYKDVDKAPFNGMTGCGNT

SEQ ID NO: 406 - protein, 20 aa, Artificial Sequence
  Lolium perenne pollen allergen epitope
GAGPKDNGGACGYKDVDKAP

SEQ ID NO: 407 - protein, 20 aa, Artificial Sequence
  Lolium perenne pollen allergen epitope
SEVEDVIPEGWKADTSYSAK

SEQ ID NO: 408 - protein, 20 aa, Artificial Sequence
  Lolium perenne pollen allergen epitope
VEKGSNPNYLAILVKYVDGD

SEQ ID NO: 409 - protein, 20 aa, Artificial Sequence
  Lolium perenne pollen allergen epitope
YPDDTKPTFHVEKGSNPNYL

SEQ ID NO: 410 - protein, 16 aa, Artificial Sequence
  Ambrosia artemisiifolia Pollen allergen Amb a 1.1 precursor epitope
GAGDENIEDRGMLATV

SEQ ID NO: 411 - protein, 16 aa, Artificial Sequence
  Ambrosia artemisiifolia Pollen allergen Amb a 1.1 precursor epitope
GAGDENIEDRGMLATV

SEQ ID NO: 412 - protein, 16 aa, Artificial Sequence
  Ambrosia artemisiifolia Pollen allergen Amb a 2 precursor epitope
GASDTHFQDLKMHVTL

SEQ ID NO: 413 - protein, 16 aa, Artificial Sequence
  Ambrosia artemisiifolia Pollen allergen Amb a 2 precursor epitope
GASDTHFQDLKMHVTL

SEQ ID NO: 414 - protein, 11 aa, Artificial Sequence
  Ambrosia artemisiifolia var. elatior Pollen allergen Amb a 3 epitope
EEAYHACDIKD

SEQ ID NO: 415 - protein, 15 aa, Artificial Sequence
  Ambrosia artemisiifolia var. elatior Pollen allergen Amb a 3 epitope
GKVYLVGGPELGGWK

SEQ ID NO: 416 - protein, 15 aa, Artificial Sequence
  Ambrosia artemisiifolia var. elatior Pollen allergen Amb a 3 epitope
LGGWKLQSDPRAYAL

SEQ ID NO: 417 - protein, 15 aa, Artificial Sequence
  Ambrosia artemisiifolia var. elatior Pollen allergen Amb a 3 epitope
PGGPDRFTLLTPGSH

SEQ ID NO: 418 - protein, 15 aa, Artificial Sequence
  Ambrosia artemisiifolia var. elatior Pollen allergen Amb a 5 epitope
AYCCSDPGRYCPWQV

SEQ ID NO: 419 - protein, 20 aa, Artificial Sequence
  Ambrosia artemisiifolia var. elatior Pollen allergen Amb a 5 epitope
CGEKRAYCCSDPGRYCPWQV

SEQ ID NO: 420 - protein, 17 aa, Artificial Sequence
  Ambrosia artemisiifolia var. elatior Pollen allergen Amb a 5 epitope
DPGRYCPWQVVCYESSE

SEQ ID NO: 421 - protein, 20 aa, Artificial Sequence
  Ambrosia artemisiifolia var. elatior Pollen allergen Amb a 5 epitope
DPGRYCPWQVVCYESSEICS

SEQ ID NO: 422 - protein, 15 aa, Artificial Sequence
  Ambrosia artemisiifolia var. elatior Pollen allergen Amb a 5 epitope
GNVCGEKRAYCCSDP

SEQ ID NO: 423 - protein, 15 aa, Artificial Sequence
  Ambrosia artemisiifolia var. elatior Pollen allergen Amb a 5 epitope
LVPCAWAGNVCGEKR

SEQ ID NO: 424 - protein, 20 aa, Artificial Sequence
  Ambrosia artemisiifolia var. elatior Pollen allergen Amb a 5 epitope
LVPCAWAGNVCGEKRAYCCS

SEQ ID NO: 425 - protein, 15 aa, Artificial Sequence
  Ambrosia artemisiifolia var. elatior Pollen allergen Amb a 5 epitope
VCYESSEICSKKCGK

SEQ ID NO: 426 - protein, 20 aa, Artificial Sequence
  Ambrosia trifida Pollen allergen Amb t 5 precursor epitope
CGKVGKYCCSPIGKYCVCYD

SEQ ID NO: 427 - protein, 20 aa, Artificial Sequence
  Ambrosia trifida Pollen allergen Amb t 5 precursor epitope
DDGLCYEGTNCGKVGKYCCS

SEQ ID NO: 428 - protein, 12 aa, Artificial Sequence
  Ambrosia trifida Pollen allergen Amb t 5 precursor epitope
GKYCVCYDSKAI

SEQ ID NO: 429 - protein, 14 aa, Artificial Sequence
  Ambrosia trifida Pollen allergen Amb t 5 precursor epitope
PIGKYCVCYDSKAI

SEQ ID NO: 430 - protein, 20 aa, Artificial Sequence
  Ambrosia trifida Pollen allergen Amb t 5 precursor epitope
PIGKYCVCYDSKAICNKNCT

SEQ ID NO: 431 - protein, 14 aa, Artificial Sequence
  Ambrosia trifida Pollen allergen Amb t 5 precursor epitope
VCYDSKAICNKNCT

SEQ ID NO: 432 - protein, 15 aa, Artificial Sequence
  Betula pendula pollen allergen Bet v 1 epitope
HEVKAEQVKATKEMG

SEQ ID NO: 433 - protein, 20 aa, Artificial Sequence
  Poa pratensis Pollen allergen KBG 60 precursor epitope
AANKYKTFVATFGAASNKAF

SEQ ID NO: 434 - protein, 20 aa, Artificial Sequence
  Poa pratensis Pollen allergen KBG 60 precursor epitope
AAPANDKFTVFEAAFNDAIK

SEQ ID NO: 435 - protein, 20 aa, Artificial Sequence
  Poa pratensis Pollen allergen KBG 60 precursor epitope
AAVDSSKAALTSKLDAAYKL

SEQ ID NO: 436 - protein, 20 aa, Artificial Sequence
  Poa pratensis Pollen allergen KBG 60 precursor epitope
AEEVKATPAGELQVIDKVDA

SEQ ID NO: 437 - protein, 20 aa, Artificial Sequence
  Poa pratensis Pollen allergen KBG 60 precursor epitope
AFKVAATAANAAPANDKFTV

SEQ ID NO: 438 - protein, 20 aa, Artificial Sequence
  Lolium perenne Pollen allergen Lol p 1 precursor epitope
AFGSMAKKGEEQNVRSAGEL

SEQ ID NO: 439 - protein, 20 aa, Artificial Sequence
  Lolium perenne Pollen allergen Lol p 1 precursor epitope
AGELELQFRRVKCKYPDDTK

SEQ ID NO: 440 - protein, 20 aa, Artificial Sequence
  Lolium perenne Pollen allergen Lol p 1 precursor epitope
AKSTWYGKPTGAGPKDNGGA

SEQ ID NO: 441 - protein, 20 aa, Artificial Sequence
  Lolium perenne Pollen allergen Lol p 1 precursor epitope
APYHFDLSGHAFGSMAKKGE

SEQ ID NO: 442 - protein, 12 aa, Artificial Sequence
  Lolium perenne Pollen allergen Lol p 1 precursor epitope
IAPYHFDLSGHA

SEQ ID NO: 443 - protein, 20 aa, Artificial Sequence
  Lolium perenne Pollen allergen Lol p VA precursor epitope
AALTKAITAMTQAQKAGKPA

SEQ ID NO: 444 - protein, 20 aa, Artificial Sequence
  Lolium perenne Pollen allergen Lol p VA precursor epitope
AANAAPTNDKFTVFESAFNK

SEQ ID NO: 445 - protein, 20 aa, Artificial Sequence
  Lolium perenne Pollen allergen Lol p VA precursor epitope
ADKFKIFEAAFSESSKGLLA

SEQ ID NO: 446 - protein, 20 aa, Artificial Sequence
  Lolium perenne Pollen allergen Lol p VA precursor epitope
AFSESSKGLLATSAAKAPGL

SEQ ID NO: 447 - protein, 20 aa, Artificial Sequence
  Lolium perenne Pollen allergen Lol p VA precursor epitope
AYAATVAAAPEVKYAVFEAA

SEQ ID NO: 448 - protein, 12 aa, Artificial Sequence
  Phleum pratense Pollen allergen Phl p 1 epitope
ACSGEPVVVHIT

SEQ ID NO: 449 - protein, 12 aa, Artificial Sequence
  Phleum pratense Pollen allergen Phl p 1 epitope
AEDVIPEGWKAD

SEQ ID NO: 450 - protein, 12 aa, Artificial Sequence
  Phleum pratense Pollen allergen Phl p 1 epitope
AGELELQFRRVK

SEQ ID NO: 451 - protein, 12 aa, Artificial Sequence
  Phleum pratense Pollen allergen Phl p 1 epitope
DKWIELKESWGA

SEQ ID NO: 452 - protein, 12 aa, Artificial Sequence
  Phleum pratense Pollen allergen Phl p 1 epitope
DKWLDAKSTWYG

SEQ ID NO: 453 - protein, 12 aa, Artificial Sequence
  Phleum pratense Pollen allergen Phl p 1 precursor epitope
FEIKCTKPEACS

SEQ ID NO: 454 - protein, 12 aa, Artificial Sequence
  Phleum pratense Pollen allergen Phl p 1 precursor epitope
YHFDLSGHAFGA

SEQ ID NO: 455 - protein, 15 aa, Artificial Sequence
  Phleum pratense Pollen allergen Phl p 1 precursor epitope
ELKESWGAIWRIDTP

SEQ ID NO: 456 - protein, 15 aa, Artificial Sequence
  Phleum pratense Pollen allergen Phl p 1 precursor epitope
EPIAPYHFDLSGHAF

SEQ ID NO: 457 - protein, 15 aa, Artificial Sequence
  Phleum pratense Pollen allergen Phl p 1 precursor epitope
FEIKCTKPEACSGEP

SEQ ID NO: 458 - protein, 15 aa, Artificial Sequence
  Phleum pratense Pollen allergen Phl p 1 precursor epitope
WGAIWRIDTPDKLTG

SEQ ID NO: 459 - protein, 15 aa, Artificial Sequence
  Phleum pratense Pollen allergen Phl p 11 epitope
RYANPIAFFRKEPLK

SEQ ID NO: 460 - protein, 15 aa, Artificial Sequence
  Phleum pratense Pollen allergen Phl p 2 epitope
EHGSDEWVAMTKGEG

SEQ ID NO: 461 - protein, 15 aa, Artificial Sequence
  Phleum pratense Pollen allergen Phl p 2 epitope
EWVAMTKGEGGVWTF

SEQ ID NO: 462 - protein, 15 aa, Artificial Sequence
  Phleum pratense Pollen allergen Phl p 2 epitope
GVWTFDSEEPLQGPF

SEQ ID NO: 463 - protein, 15 aa, Artificial Sequence
  Phleum pratense Pollen allergen Phl p 2 epitope
KNVFDDVVPEKYTIG

SEQ ID NO: 464 - protein, 15 aa, Artificial Sequence
  Phleum pratense Pollen allergen Phl p 2 epitope
LQGPFNFRFLTEKGM

SEQ ID NO: 465 - protein, 15 aa, Artificial Sequence
  Phleum pratense Pollen allergen Phl p 4 epitope
FKPFAEYKSDYVYEP

SEQ ID NO: 466 - protein, 15 aa, Artificial Sequence
  Phleum pratense Pollen allergen Phl p 4 epitope
FPKEVWEQIFSTWLL

SEQ ID NO: 467 - protein, 15 aa, Artificial Sequence
  Phleum pratense Pollen allergen Phl p 4 epitope
FVHLGHRDNIEDDLL

SEQ ID NO: 468 - protein, 15 aa, Artificial Sequence
  Phleum pratense Pollen allergen Phl p 4 epitope
GIVVAWKVRLLPVPP

SEQ ID NO: 469 - protein, 15 aa, Artificial Sequence
  Phleum pratense Pollen allergen Phl p 4 epitope
NRNNTFKPFAEYKSD

SEQ ID NO: 470 - protein, 12 aa, Artificial Sequence
  Phleum pratense Pollen allergen Phl p 5a epitope
EVKYTVFETALK

SEQ ID NO: 471 - protein, 19 aa, Artificial Sequence
  Phleum pratense Pollen allergen Phl p 5a epitope
NAGFKAALAGAGVQPADKY

SEQ ID NO: 472 - protein, 27 aa, Artificial Sequence
  Phleum pratense Pollen allergen Phl p 5b precursor epitope
AAGKATTEEQKLIEDINVGFKAAVAAA

SEQ ID NO: 473 - protein, 33 aa, Artificial Sequence
  Phleum pratense Pollen allergen Phl p 5b precursor epitope
AAGKATTEEQKLIEDINVGFKAAVAAAASVPAA

SEQ ID NO: 474 - protein, 19 aa, Artificial Sequence
  Phleum pratense Pollen allergen Phl p 5b precursor epitope
AAVAAAASVPAADKFKTFE

SEQ ID NO: 475 - protein, 27 aa, Artificial Sequence
  Phleum pratense Pollen allergen Phl p 5b precursor epitope
AKFDSFVASLTEALRVIAGALEVHAVK

SEQ ID NO: 476 - protein, 19 aa, Artificial Sequence
  Phleum pratense Pollen allergen Phl p 5b precursor epitope
AMSEVQKVSQPATGAATVA

SEQ ID NO: 477 - protein, 20 aa, Artificial Sequence
  Chamaecyparis obtusa Polygalacturonase epitope
ARWKNSKIWLQFAQLTDFNL

SEQ ID NO: 478 - protein, 20 aa, Artificial Sequence
  Chamaecyparis obtusa Polygalacturonase epitope
AVLLVPANKKFFVNNLVFRG

SEQ ID NO: 479 - protein, 20 aa, Artificial Sequence
  Chamaecyparis obtusa Polygalacturonase epitope
DGTIVAQPDPARWKNSKIWL

SEQ ID NO: 480 - protein, 20 aa, Artificial Sequence
  Chamaecyparis obtusa Polygalacturonase epitope
FFVNNLVFRGPCQPHLSFKV

SEQ ID NO: 481 - protein, 20 aa, Artificial Sequence
  Chamaecyparis obtusa Polygalacturonase epitope
FGECEGVKIQGLKIKAPRDS

SEQ ID NO: 482 - protein, 15 aa, Artificial Sequence
  Cryptomeria japonica Polygalacturonase precursor epitope
AAYQNPASWKNNRIW

SEQ ID NO: 483 - protein, 15 aa, Artificial Sequence
  Cryptomeria japonica Polygalacturonase precursor epitope
ACKKPSAMLLVPGNK

SEQ ID NO: 484 - protein, 15 aa, Artificial Sequence
  Cryptomeria japonica Polygalacturonase precursor epitope
AIKFDFSTGLIIQGL

SEQ ID NO: 485 - protein, 15 aa, Artificial Sequence
  Cryptomeria japonica Polygalacturonase precursor epitope
AINIFNVEKYGAVGD

SEQ ID NO: 486 - protein, 15 aa, Artificial Sequence
  Cryptomeria japonica Polygalacturonase precursor epitope
ANGYFSGHVIPACKN

SEQ ID NO: 487 - protein, 16 aa, Artificial Sequence
  Arabidopsis thaliana Probable pectate lyase 18 precursor epitope
GHSDTYSRDKNMQVTI

SEQ ID NO: 488 - protein, 15 aa, Artificial Sequence
  Phleum pratense Profilin-2/4 epitope
LGHDGTVWAQSADFP

SEQ ID NO: 489 - protein, 20 aa, Artificial Sequence
  Hevea brasiliensis Pro-hevein precursor epitope
DEYCSPDHNCQSNCKDSGEG

SEQ ID NO: 490 - protein, 20 aa, Artificial Sequence
  Hevea brasiliensis Pro-hevein precursor epitope
EQCGRQAGGKLCPNNLCCSQ

SEQ ID NO: 491 - protein, 43 aa, Artificial Sequence
  Hevea brasiliensis Pro-hevein precursor epitope
EQCGRQAGGKLCPNNLCCSQWGWCGSTDEYCSPDHNCQSNCKD

SEQ ID NO: 492 - protein, 20 aa, Artificial Sequence
  Hevea brasiliensis Pro-hevein precursor epitope
KLCPNNLCCSQWGWCGSTDE

SEQ ID NO: 493 - protein, 20 aa, Artificial Sequence
  Hevea brasiliensis Pro-hevein precursor epitope
NGGLDLDVNVFRQLDTDGKG

SEQ ID NO: 494 - protein, 10 aa, Artificial Sequence
  Prunus persica pru p 1 epitope
GKCGVSIPYK

SEQ ID NO: 495 - protein, 10 aa, Artificial Sequence
  Prunus persica pru p 1 epitope
ITCGQVSSSL

SEQ ID NO: 496 - protein, 10 aa, Artificial Sequence
  Prunus persica pru p 1 epitope
SIPYKISAST

SEQ ID NO: 497 - protein, 15 aa, Artificial Sequence
  Prunus persica pru p 1 epitope
DRQAACNCLKQLSAS

SEQ ID NO: 498 - protein, 15 aa, Artificial Sequence
  Prunus persica pru p 1 epitope
VNPNNAAALPGKCGV

SEQ ID NO: 499 - protein, 16 aa, Artificial Sequence
  Arabidopsis thaliana Putative pectate lyase 17 precursor epitope
GHNDNFVKDVKMKVTV

SEQ ID NO: 500 - protein, 16 aa, Artificial Sequence
  Homo sapiens RAD51-like 1 isoform 1 epitope
TRLILQYLDSERRQIL

SEQ ID NO: 501 - protein, 16 aa, Artificial Sequence
  Aspergillus fumigatus Ribonuclease mitogillin precursor epitope
DPGPARVIYTYPNKVF

SEQ ID NO: 502 - protein, 20 aa, Artificial Sequence
  Aspergillus fumigatus Ribonuclease mitogillin precursor epitope
ATWTCINQQLNPKTNKWEDK

SEQ ID NO: 503 - protein, 20 aa, Artificial Sequence
  Aspergillus fumigatus Ribonuclease mitogillin precursor epitope
HYLLEFPTFPDGHDYKFDSK

SEQ ID NO: 504 - protein, 20 aa, Artificial Sequence
  Aspergillus fumigatus Ribonuclease mitogillin precursor epitope
KFDSKKPKEDPGPARVIYTY

SEQ ID NO: 505 - protein, 20 aa, Artificial Sequence
  Aspergillus fumigatus Ribonuclease mitogillin precursor epitope
LIKGRTPIKFGKADCDRPPK

SEQ ID NO: 506 - protein, 20 aa, Artificial Sequence
  Aspergillus fumigatus Ribonuclease mitogillin precursor epitope
SYPHWFTNGYDGNGKLIKGR

SEQ ID NO: 507 - protein, 19 aa, Artificial Sequence
  Hevea brasiliensis Rubber elongation factor protein epitope
AEDEDNQQGQGEGLKYLGF

SEQ ID NO: 508 - protein, 19 aa, Artificial Sequence
  Hevea brasiliensis Rubber elongation factor protein epitope
FSNVYLFAKDKSGPLQPGV

SEQ ID NO: 509 - protein, 19 aa, Artificial Sequence
  Hevea brasiliensis Rubber elongation factor protein epitope
KFVDSTVVASVTIIDRSLP

SEQ ID NO: 510 - protein, 19 aa, Artificial Sequence
  Hevea brasiliensis Rubber elongation factor protein epitope
QPGVDIIEGPVKNVAVPLY

SEQ ID NO: 511 - protein, 19 aa, Artificial Sequence
  Hevea brasiliensis Rubber elongation factor protein epitope
RSLPPIVKDASIQVVSAIR

SEQ ID NO: 512 - protein, 17 aa, Artificial Sequence
  Bos taurus Serum albumin precursor epitope
DDSPDLPKLKPDPNTLC

SEQ ID NO: 513 - protein, 20 aa, Artificial Sequence
  Bos taurus Serum albumin precursor epitope
EKDAIPENLPPLTADFAEDK

SEQ ID NO: 514 - protein, 9 aa, Artificial Sequence
  Bos taurus Serum albumin precursor epitope
ESHAGCEKS

SEQ ID NO: 515 - protein, 10 aa, Artificial Sequence
  Bos taurus Serum albumin precursor epitope
HPEYAVSVLL

SEQ ID NO: 516 - protein, 9 aa, Artificial Sequence
  Bos taurus Serum albumin precursor epitope
LSLILNRLC

SEQ ID NO: 517 - protein, 12 aa, Artificial Sequence
  Hevea brasiliensis Small rubber particle protein epitope
DFVRAAGVYAVD

SEQ ID NO: 518 - protein, 12 aa, Artificial Sequence
  Hevea brasiliensis Small rubber particle protein epitope
KYLDFVRAAGVY

SEQ ID NO: 519 - protein, 12 aa, Artificial Sequence
  Hevea brasiliensis Small rubber particle protein epitope
NVVKTVVTPVYY

SEQ ID NO: 520 - protein, 12 aa, Artificial Sequence
  Hevea brasiliensis Small rubber particle protein epitope
PRIVLDVASSVF

SEQ ID NO: 521 - protein, 12 aa, Artificial Sequence
  Hevea brasiliensis Small rubber particle protein epitope
QGYRVSSYLPLL

SEQ ID NO: 522 - protein, 15 aa, Artificial Sequence
  Glycine max Stress-induced protein SAM22 epitope
ALFKAIEAYLLAHPD

SEQ ID NO: 523 - protein, 15 aa, Artificial Sequence
  Cryptomeria japonica Sugi basic protein precursor epitope
AFNVENGNATPQLTK

SEQ ID NO: 524 - protein, 15 aa, Artificial Sequence
  Cryptomeria japonica Sugi basic protein precursor epitope
ANNNYDPWTIYAIGG

SEQ ID NO: 525 - protein, 15 aa, Artificial Sequence
  Cryptomeria japonica Sugi basic protein precursor epitope
AYSDDKSMKVTVAFN

SEQ ID NO: 526 - protein, 15 aa, Artificial Sequence
  Cryptomeria japonica Sugi basic protein precursor epitope
CGQRMPRARYGLVHV

SEQ ID NO: 527 - protein, 15 aa, Artificial Sequence
  Cryptomeria japonica Sugi basic protein precursor epitope
CSNWVWQSTQDVFYN

SEQ ID NO: 528 - protein, 20 aa, Artificial Sequence
  Trichophyton rubrum Tri r 2 allergen epitope
ADFSNYGAVVDVYAPGKDIT

SEQ ID NO: 529 - protein, 20 aa, Artificial Sequence
  Trichophyton rubrum Tri r 2 allergen epitope
AKGVSLVAVKVLDCDGSGSN

SEQ ID NO: 530 - protein, 20 aa, Artificial Sequence
  Trichophyton rubrum Tri r 2 allergen epitope
ASNQAAKAISDAGIFMAVAA

SEQ ID NO: 531 - protein, 20 aa, Artificial Sequence
  Trichophyton rubrum Tri r 2 allergen epitope
DCNGHGTHVAGTVGGTKYGL

SEQ ID NO: 532 - protein, 20 aa, Artificial Sequence
  Trichophyton rubrum Tri r 2 allergen epitope
DPSAGKGVTAYIIDTGIDID

SEQ ID NO: 533 - protein, 12 aa, Artificial Sequence
  Vespula vulgaris Venom allergen 5 precursor epitope
ACKYGSLKPNCG

SEQ ID NO: 534 - protein, 12 aa, Artificial Sequence
  Vespula vulgaris Venom allergen 5 precursor epitope
CNYGPSGNFMNE

SEQ ID NO: 535 - protein, 12 aa, Artificial Sequence
  Vespula vulgaris Venom allergen 5 precursor epitope
DVAKYQVGQNVA

SEQ ID NO: 536 - protein, 12 aa, Artificial Sequence
  Vespula vulgaris Venom allergen 5 precursor epitope
EKWHKHYLVCNY

SEQ ID NO: 537 - protein, 12 aa, Artificial Sequence
  Vespula vulgaris Venom allergen 5 precursor epitope
ELAYVAQVWANQ

SEQ ID NO: 538 - protein, 15 aa, Artificial Sequence
  Corylus avellana 11S globulin-like protein epitope
AFQISREEARRLKYN

SEQ ID NO: 539 - protein, 12 aa, Artificial Sequence
  Carya illinoinensis 11S legumin protein epitope
EESQRQSQQGQR

SEQ ID NO: 540 - protein, 18 aa, Artificial Sequence
  Fagopyrum esculentum 13S globulin epitope
DAHQPTRRVRKGDVVALP

SEQ ID NO: 541 - protein, 12 aa, Artificial Sequence
  Fagopyrum esculentum 13S globulin seed storage protein 1 precursor (Legumin-like protein 1) epitope
FKQNVNRPSRAD

SEQ ID NO: 542 - protein, 12 aa, Artificial Sequence
  Fagopyrum esculentum 13S globulin seed storage protein 3 precursor (Legumin-like protein 3) (Allergen Fag e 1) epitope
DISTKEAFRLKN

SEQ ID NO: 543 - protein, 12 aa, Artificial Sequence
  Anacardium occidentale 2s albumin epitope
CQRQFEEQQRFR

SEQ ID NO: 544 - protein, 10 aa, Artificial Sequence
  Sesamum indicum 2S seed storage protein 1 epitope
HFRECCNEIR

SEQ ID NO: 545 - protein, 10 aa, Artificial Sequence
  Sesamum indicum 2S seed storage protein 1 precursor epitope
CMQWMRSMRG

SEQ ID NO: 546 - protein, 14 aa, Artificial Sequence
  Bertholletia excelsa 2S sulfur-rich seed storage protein precursor (Allergen Ber e 1) epitope
CRCEGLRMMMMRMQ

SEQ ID NO: 547 - protein, 40 aa, Artificial Sequence
  Homo sapiens 52 kDa Ro protein epitope
LEKDEREQLRILGEKEAKLAQQSQALQELISELDRRCHSS

SEQ ID NO: 548 - protein, 10 aa, Artificial Sequence
  Homo sapiens 52-kD SS-A/Ro autoantigen epitope
QEKLQVALGE

SEQ ID NO: 549 - protein, 21 aa, Artificial Sequence
  Homo sapiens 5-hydroxytryptamine (serotonin) receptor 4 epitope
GIIDLIEKRKFNQNSNSTYCV

SEQ ID NO: 550 - protein, 10 aa, Artificial Sequence
  Homo sapiens 60 kDa heat shock protein, mitochondrial precursor epitope
DGVAVLKVGG

SEQ ID NO: 551 - protein, 22 aa, Artificial Sequence
  Homo sapiens 60 kDa SS-A/Ro ribonucleoprotein epitope
ELYKEKALSVETEKLLKYLEAV

SEQ ID NO: 552 - protein, 22 aa, Artificial Sequence
  Homo sapiens 60S acidic ribosomal protein P0 epitope
AKVEAKEESEESDEDMGFGLFD

SEQ ID NO: 553 - protein, 13 aa, Artificial Sequence
  Homo sapiens 60S acidic ribosomal protein P2 epitope
EESDDDMGFGLFD

SEQ ID NO: 554 - protein, 50 aa, Artificial Sequence
  Homo sapiens 64 Kd autoantigen epitope
ATKKEEEKKGGDRNTGLSRDKDKKREEMKEVAKKEDDEKVKGERRNTDTR

SEQ ID NO: 555 - protein, 19 aa, Artificial Sequence
  Homo sapiens 65 kDa heat shock protein epitope
ALLRCIPALDSLTPANEDC

SEQ ID NO: 556 - protein, 14 aa, Artificial Sequence
  Homo sapiens Acetylcholine receptor subunit alpha precursor epitope
AINPESDQPDLSNF

SEQ ID NO: 557 - protein, 21 aa, Artificial Sequence
  Cynodon dactylon acidic Cyn d 1 isoallergen isoform 1 precursor epitope
QDDVIPEDWKPDTVYKSKIQF

SEQ ID NO: 558 - protein, 50 aa, Artificial Sequence
  Cynodon dactylon acidic Cyn d 1 isoallergen isoform 3 precursor epitope
EEDKLRKAGELMLQFRRVKCEYPSDTKITFHVEKGSSPNYLALLVKYAAG

SEQ ID NO: 559 - protein, 8 aa, Artificial Sequence
  Homo sapiens acidic ribosomal phosphoprotein (P0) epitope
AAAAAPAK

SEQ ID NO: 560 - protein, 15 aa, Artificial Sequence
  Homo sapiens acidic ribosomal phosphoprotein (P1) epitope
ESEESDDDMGFGLFD

SEQ ID NO: 561 - protein, 15 aa, Artificial Sequence
  Homo sapiens acidic ribosomal phosphoprotein (P2) epitope
APAAGSAPAAAEEKK

SEQ ID NO: 562 - protein, 16 aa, Artificial Sequence
  Homo sapiens Adrenergic, beta-2-, receptor, surface epitope
HWYRATHQEAINCYAN

SEQ ID NO: 563 - protein, 10 aa, Artificial Sequence
  Homo sapiens Alanyl-tRNA synthetase, cytoplasmic epitope
FIDEPRRRPI

SEQ ID NO: 564 - protein, 7 aa, Artificial Sequence
  Bos taurus albumin epitope
PVESKVT

SEQ ID NO: 565 - protein, 13 aa, Artificial Sequence
  Juglans regia Albumin seed storage protein epitope
GLRGEEMEEMVQS

SEQ ID NO: 566 - protein, 18 aa, Artificial Sequence
  Cochliobolus lunatus alcohol dehydrogenase epitope
AVNGDWPLPTKLPLVGGH

SEQ ID NO: 567 - protein, 37 aa, Artificial Sequence
  Penicillium chrysogenum alkaline serine protease epitope
ANVVQRNAPSWGLSRISSKKSGATDYVYDSTAGEGIV

SEQ ID NO: 568 - protein, 10 aa, Artificial Sequence
  Arachis hypogaea allergen epitope
DDQCQRQLQR

SEQ ID NO: 569 - protein, 15 aa, Artificial Sequence
  Anacardium occidentale allergen Ana o 2 epitope
EESEDEKRRWGQRDN

SEQ ID NO: 570 - protein, 10 aa, Artificial Sequence
  Arachis hypogaea Allergen Ara h 1, clone P41B precursor epitope
AKSSPYQKKT

SEQ ID NO: 571 - protein, 15 aa, Artificial Sequence
  Arachis hypogaea allergen Arah3/Arah4 epitope
AGVALSRLVLRRNAL

SEQ ID NO: 572 - protein, 10 aa, Artificial Sequence
  Arachis hypogaea allergen Arah6 epitope
DRQMVQHFKR

SEQ ID NO: 573 - protein, 11 aa, Artificial Sequence
  Periplaneta americana Allergen Cr-PI epitope
IPKGKKGGQAY

SEQ ID NO: 574 - protein, 8 aa, Artificial Sequence
  Aspergillus fumigatus allergen I/a; Asp f I/a epitope
INQQLNPK

SEQ ID NO: 575 - protein, 10 aa, Artificial Sequence
  Arachis hypogaea Allergen II epitope
DRLQGRQQEQ

SEQ ID NO: 576 - protein, 15 aa, Artificial Sequence
  Lens culinaris allergen Len c 1.0101 epitope
AINASSDLNLIGFGI

SEQ ID NO: 577 - protein, 12 aa, Artificial Sequence
  Dermatophagoides farinae Allergen Mag epitope
DVELSLRSSDIA

SEQ ID NO: 578 - protein, 31 aa, Artificial Sequence
  Penicillium chrysogenum Allergen Pen n 18 epitope
AHIKKSKKGDKKFKGSVANMSLGGGSSRTLD

SEQ ID NO: 579 - protein, 14 aa, Artificial Sequence
  Sinapis alba Allergen Sin a 1 epitope
QGPHVISRIYQTAT

SEQ ID NO: 580 - protein, 12 aa, Artificial Sequence
  Ziziphus mauritiana allergen Ziz m 1 epitope
KTNYSSSIILEY

SEQ ID NO: 581 - protein, 37 aa, Artificial Sequence
  Fagopyrum tataricum allergenic protein epitope
DISTEEAYKLKNGRQEVEVFRPFQSRYEKEEEKERER

SEQ ID NO: 582 - protein, 14 aa, Artificial Sequence
  Homo sapiens alpha 2 interferon epitope
EVVRAEIMRSFSLS

SEQ ID NO: 583 - protein, 30 aa, Artificial Sequence
  Bos taurus alpha S1 casein epitope
EDQAMEDIKQMEAESISSSEEIVPNSVEQK

SEQ ID NO: 584 - protein, 10 aa, Artificial Sequence
  Triticum aestivum Alpha/beta-gliadin A-II precursor epitope
QVSFQQPQQQ

SEQ ID NO: 585 - protein, 10 aa, Artificial Sequence
  Triticum aestivum Alpha/beta-gliadin A-V epitope
LALQTLPAMC

SEQ ID NO: 586 - protein, 10 aa, Artificial Sequence
  Homo sapiens alpha-1 type IV collagen epitope
SRCQVCMRRT

SEQ ID NO: 587 - protein, 12 aa, Artificial Sequence
  Homo sapiens alpha1A-voltage-dependent calcium channel epitope
EDSDEDEFQITE

SEQ ID NO: 588 - protein, 15 aa, Artificial Sequence
  Homo sapiens alpha-2 type XI collagen epitope
GSLDSLRREIEQMRR

SEQ ID NO: 589 - protein, 20 aa, Artificial Sequence
  Bos taurus alpha2(I) collagen epitope
LPGLKGHNGLQGLPGLAGHH

SEQ ID NO: 590 - protein, 5 aa, Artificial Sequence
  Triticum aestivum Alpha-amylase inhibitor 0.28 precursor (CIII) (WMAI-1) epitope
AYPDV

SEQ ID NO: 591 - protein, 17 aa, Artificial Sequence
  Homo sapiens Alpha-enolase epitope
KIHAREIFDSRGNPTVE

SEQ ID NO: 592 - protein, 15 aa, Artificial Sequence
  Homo sapiens alpha-fibrinogen precursor epitope
GPRVVERHQSACKDS

SEQ ID NO: 593 - protein, 12 aa, Artificial Sequence
  Triticum aestivum Alpha-gliadin epitope
LGQGSFRPSQQN

SEQ ID NO: 594 - protein, 10 aa, Artificial Sequence
  Bos taurus Alpha-lactalbumin epitope
KDLKGYGGVS

SEQ ID NO: 595 - protein, 14 aa, Artificial Sequence
  Bos taurus Alpha-lactalbumin precursor epitope
KCEVFRELKDLKGY

SEQ ID NO: 596 - protein, 20 aa, Artificial Sequence
  Bos taurus alpha-S1-casein epitope
LNENLLRFFVAPFPQVFGKE

SEQ ID NO: 597 - protein, 10 aa, Artificial Sequence
  Bos taurus Alpha-S1-casein precursor epitope
AMEDIKQMEA

SEQ ID NO: 598 - protein, 10 aa, Artificial Sequence
  Bos taurus Alpha-S2-casein precursor epitope
ENLCSTFCKE

SEQ ID NO: 599 - protein, 7 aa, Artificial Sequence
  Homo sapiens anti-beta-amyloid peptide immunoglobulin heavy chain variable region epitope
AHIWWND

SEQ ID NO: 600 - protein, 24 aa, Artificial Sequence
  Homo sapiens Aquaporin-4 epitope
FCPDVEFKRRFKEAFSKAAQQTKG

SEQ ID NO: 601 - protein, 15 aa, Artificial Sequence
  Arachis hypogaea Ara h 2.01 allergen epitope
CCNELNEFENNQRCM

SEQ ID NO: 602 - protein, 20 aa, Artificial Sequence
  Homo sapiens ATP-dependent DNA helicase 2 subunit 2 epitope
EEASGSSVTAEEAKKFLAPK

SEQ ID NO: 603 - protein, 28 aa, Artificial Sequence
  Homo sapiens autoantigen epitope
EIRVRLQSASPSTRWTELDDVKRLLKGS

SEQ ID NO: 604 - protein, 16 aa, Artificial Sequence
  Homo sapiens Band 3 anion transport protein epitope
LFKPPKYHPDVPYVKR

SEQ ID NO: 605 - protein, 15 aa, Artificial Sequence
  Glycine max Bd 30K (34 kDa maturing seed protein) epitope
EDWGEDGYIWIQRNT

SEQ ID NO: 606 - protein, 7 aa, Artificial Sequence
  Homo sapiens Bence Jones protein HAG epitope
AWHQQQP

SEQ ID NO: 607 - protein, 8 aa, Artificial Sequence
  Betula pendula Bet v 4 epitope
FARANRGL

SEQ ID NO: 608 - protein, 9 aa, Artificial Sequence
  Musa acuminata beta-1, 3-glucananse epitope
GLFYPNKQP

SEQ ID NO: 609 - protein, 15 aa, Artificial Sequence
  Hevea brasiliensis beta-1,3-glucanase epitope
GLFFPDKRPKYNLNF

SEQ ID NO: 610 - protein, 12 aa, Artificial Sequence
  Olea europaea beta-1,3-glucanase-like protein epitope
AGRNSWNCDFSQ

SEQ ID NO: 611 - protein, 6 aa, Artificial Sequence
  Homo sapiens beta-2-glycoprotein 1 precursor epitope
LKTPRV

SEQ ID NO: 612 - protein, 6 aa, Artificial Sequence
  Homo sapiens beta-2-glycoprotein I epitope
TLRVYK

SEQ ID NO: 613 - protein, 13 aa, Artificial Sequence
  Bos taurus beta-casein epitope
QSKVLPVPQKAVP

SEQ ID NO: 614 - protein, 12 aa, Artificial Sequence
  Bos taurus Beta-casein precursor epitope
DELQDKIHPFAQ

SEQ ID NO: 615 - protein, 10 aa, Artificial Sequence
  Bos taurus Beta-lactoglobulin epitope
AQKKIIAEKT

SEQ ID NO: 616 - protein, 16 aa, Artificial Sequence
  Bos taurus Beta-lactoglobulin precursor epitope
AASDISLLDAQSAPLR

SEQ ID NO: 617 - protein, 7 aa, Artificial Sequence
  Homo sapiens Botulinum neurotoxin type E epitope
WKAPSSP

SEQ ID NO: 618 - protein, 19 aa, Artificial Sequence
  Homo sapiens bullous pemphigoid antigen epitope
KSTAKDCTFKPDFEMTVKE

SEQ ID NO: 619 - protein, 20 aa, Artificial Sequence
  Homo sapiens Bullous pemphigoid antigen 1, isoforms 1/2/3/4/5/8 epitope
LTDTKTGLHFNINEAIEQGT

SEQ ID NO: 620 - protein, 8 aa, Artificial Sequence
  Fagopyrum esculentum BW 16kDa allergen epitope
EGVRDLKE

SEQ ID NO: 621 - protein, 17 aa, Artificial Sequence
  Homo sapiens calcium channel, alpha 1A subunit isoform 3 epitope
GNIGIDVEDEDSDEDEF

SEQ ID NO: 622 - protein, 15 aa, Artificial Sequence
  Homo sapiens Calpastatin epitope
AVCRTSMCSIQSAPP

SEQ ID NO: 623 - protein, 18 aa, Artificial Sequence
  Homo sapiens Calreticulin precursor epitope
KEQFLDGDGWTSRWIESK

SEQ ID NO: 624 - protein, 13 aa, Artificial Sequence
  Homo sapiens Ca-sensing receptor epitope
FVAQNKIDSLNLD

SEQ ID NO: 625 - protein, 9 aa, Artificial Sequence
  Homo sapiens Caspase-8 precursor epitope
DRNGTHLDA

SEQ ID NO: 626 - protein, 14 aa, Artificial Sequence
  Homo sapiens centromere protein A isoform a epitope
GPSRRGPSLGASSH

SEQ ID NO: 627 - protein, 10 aa, Artificial Sequence
  Homo sapiens centromere protein B, 80kDa epitope
MGPKRRQLTF

SEQ ID NO: 628 - protein, 10 aa, Artificial Sequence
  Homo sapiens centromere protein-A epitope
EAPRRRSPSP

SEQ ID NO: 629 - protein, 17 aa, Artificial Sequence
  Betula pendula Chain A, Birch Pollen Profilin epitope
AQSSSFPQFKPQEITGI

SEQ ID NO: 630 - protein, 5 aa, Artificial Sequence
  Homo sapiens Chain A, Crystal Structure Of The Glycosylated Five-Domain Human Beta2-Glycoprotein I Purified From Blood Plasma epitope
RGGMR

SEQ ID NO: 631 - protein, 7 aa, Artificial Sequence
  Homo sapiens Chain H, Three-Dimensional Structure Of A Human Immunoglobulin With A Hinge Deletion epitope
ALPAPIE

SEQ ID NO: 632 - protein, 27 aa, Artificial Sequence
  Homo sapiens cholesterol side-chain cleavage enzyme P450scc (EC 1.14.15.67) epitope
FDPENFDPTRWLSKDKNITYFRNLGFG

SEQ ID NO: 633 - protein, 10 aa, Artificial Sequence
  Homo sapiens citrate synthase epitope
ALKHLPNDPM

SEQ ID NO: 634 - protein, 5 aa, Artificial Sequence
  Homo sapiens claudin 11 epitope
AHRET

SEQ ID NO: 635 - protein, 11 aa, Artificial Sequence
  Homo sapiens Coagulation factor VIII precursor epitope
APDDRSYKSQY

SEQ ID NO: 636 - protein, 20 aa, Artificial Sequence
  Oncorhynchus mykiss collagen a2(I) epitope
MKGLRGHGGLQGMPGPNGPS

SEQ ID NO: 637 - protein, 14 aa, Artificial Sequence
  Homo sapiens Collagen alpha-1(II) chain epitope
ARGAQGPPGATGFP

SEQ ID NO: 638 - protein, 8 aa, Artificial Sequence
  Homo sapiens collagen alpha-1(VII) chain precursor epitope
GTLHVVQR

SEQ ID NO: 639 - protein, 23 aa, Artificial Sequence
  Homo sapiens Collagen alpha-1(XVII) chain epitope
RSILPYGDSMDRIEKDRLQGMAP

SEQ ID NO: 640 - protein, 15 aa, Artificial Sequence
  Homo sapiens Collagen alpha-3(IV) chain epitope
TAIPSCPEGTVPLYS

SEQ ID NO: 641 - protein, 8 aa, Artificial Sequence
  Homo sapiens collagen VII epitope
IIWRSTQG

SEQ ID NO: 642 - protein, 46 aa, Artificial Sequence
  Bos taurus collagen, type I, alpha 2 epitope
APGPDGNNGAQGPPGLQGVQGGKGEQGPAGPPGFQGLPGPAGTAGE

SEQ ID NO: 643 - protein, 9 aa, Artificial Sequence
  Homo sapiens collagen, type II, alpha 1 epitope
PPGPTGASG

SEQ ID NO: 644 - protein, 11 aa, Artificial Sequence
  Homo sapiens collagen, type II, alpha 1 isoform 1 precursor epitope
ARGLTGRPGDA

SEQ ID NO: 645 - protein, 11 aa, Artificial Sequence
  Homo sapiens collagen, type II, alpha 1 isoform 2 precursor epitope
LVGPRGERGFP

SEQ ID NO: 646 - protein, 9 aa, Artificial Sequence
  Homo sapiens Complement C1q subcomponent subunit A epitope
KGEQGEPGA

SEQ ID NO: 647 - protein, 10 aa, Artificial Sequence
  Homo sapiens Condensin-2 complex subunit D3 epitope
PTPETGPLQR

SEQ ID NO: 648 - protein, 15 aa, Artificial Sequence
  Arachis hypogaea Conglutin-7 precursor epitope
AAHASARQQWELQGD

SEQ ID NO: 649 - protein, 8 aa, Artificial Sequence
  Periplaneta americana Cr-PII allergen epitope
IRSWFGLP

SEQ ID NO: 650 - protein, 11 aa, Artificial Sequence
  Cochliobolus lunatus Cytochrome c epitope
ENPKKYIPGTK

SEQ ID NO: 651 - protein, 10 aa, Artificial Sequence
  Rattus norvegicus Cytochrome P450 3A1 epitope
DMVLNETLRL

SEQ ID NO: 652 - protein, 15 aa, Artificial Sequence
  Homo sapiens cytoskeleton-associated protein 5 isoform b epitope
CQALVRMLAKKPGWK

SEQ ID NO: 653 - protein, 9 aa, Artificial Sequence
  Dermatophagoides farinae Der f 2 epitope
IATHAKIRD

SEQ ID NO: 654 - protein, 15 aa, Artificial Sequence
  Dermatophagoides farinae Der f 7 allergen epitope
HIGGLSILDPIFGVL

SEQ ID NO: 655 - protein, 43 aa, Artificial Sequence
  Dermatophagoides pteronyssinus Der p 1 allergen epitope
AREQSCRRPNAQRFGISNYCQIYPPNANKIREALAQTHSAIAV

SEQ ID NO: 656 - protein, 15 aa, Artificial Sequence
  Dermatophagoides pteronyssinus Der p 7 allergen polypeptide epitope
HIGGLSILDPIFAVL

SEQ ID NO: 657 - protein, 12 aa, Artificial Sequence
  Homo sapiens Desmoglein-1 epitope
REWIKFAAACRE

SEQ ID NO: 658 - protein, 12 aa, Artificial Sequence
  Homo sapiens Desmoglein-3 precursor epitope
REWVKFAKPCRE

SEQ ID NO: 659 - protein, 30 aa, Artificial Sequence
  Homo sapiens desmoglein-3 preproprotein epitope
SQEPAGTPMFLLSRNTGEVRTLTNSLDREQ

SEQ ID NO: 660 - protein, 12 aa, Artificial Sequence
  Homo sapiens desmoplakin epitope
GNSSYSYSYSFS

SEQ ID NO: 661 - protein, 20 aa, Artificial Sequence
  Homo sapiens desmoplakin isoform II epitope
LVDRKTGSQYDIQDAIDKGL

SEQ ID NO: 662 - protein, 18 aa, Artificial Sequence
  Homo sapiens dihydrolipoamide S-acetyltransferase (E2 component of pyruvate dehydrogenase complex), isoform CRA_a epitope
AEIETDKATIGFEVQEEG

SEQ ID NO: 663 - protein, 17 aa, Artificial Sequence
  Homo sapiens DNA topoisomerase 1 epitope
GVPIEKIYNKTQREKFA

SEQ ID NO: 664 - protein, 20 aa, Artificial Sequence
  Homo sapiens DNA topoisomerase I epitope
ELDGQEYVVEFDFLGKDSIR

SEQ ID NO: 665 - protein, 20 aa, Artificial Sequence
  Homo sapiens DNA topoisomerase II beta epitope
HPMLPNYKNFKGTIQELGQN

SEQ ID NO: 666 - protein, 7 aa, Artificial Sequence
  Homo sapiens DNA-directed RNA polymerase II subunit RPB1 epitope
YSPTSPS

SEQ ID NO: 667 - protein, 36 aa, Artificial Sequence
  Homo sapiens E3 ubiquitin-protein ligase TRIM9 isoform 2 epitope
AFNKTGVSPYSKTLVLQTSEGKALQQYPSERELRGI

SEQ ID NO: 668 - protein, 39 aa, Artificial Sequence
  Candida albicans Enolase 1 (2-phosphoglycerate dehydratase) (2-phospho-D-glycerate hydro-lyase) epitope
QAANDSYAAGWGVMVSHRSGETEDTFIADLSVGLRSGQI

SEQ ID NO: 669 - protein, 16 aa, Artificial Sequence
  Homo sapiens enolase 1 variant epitope
KIHAREIFDSRGNPTV

SEQ ID NO: 670 - protein, 21 aa, Artificial Sequence
  Hevea brasiliensis ENSP-like protein epitope
FPLITCCGYGGKYNFSVTAPC

SEQ ID NO: 671 - protein, 20 aa, Artificial Sequence
  Homo sapiens envoplakin epitope
AGETKPSSSLSIGSIISKSP

SEQ ID NO: 672 - protein, 12 aa, Artificial Sequence
  Fagopyrum esculentum Fag e 1 epitope
AVVLKAGNEGLE

SEQ ID NO: 673 - protein, 3 aa, Artificial Sequence
  Homo sapiens Fas AMA epitope
CVP

SEQ ID NO: 674 - protein, 18 aa, Artificial Sequence
  Homo sapiens FGA protein epitope
SRALAREVDLKDYEDQQK

SEQ ID NO: 675 - protein, 20 aa, Artificial Sequence
  Homo sapiens FGB protein epitope
ARGHRPLDKKREEAPSLRPA

SEQ ID NO: 676 - protein, 19 aa, Artificial Sequence
  Homo sapiens fibrin beta epitope
ANKYQISVNKYRGTAGNAL

SEQ ID NO: 677 - protein, 15 aa, Artificial Sequence
  Homo sapiens fibrinogen alpha chain isoform alpha preproprotein epitope
DSPGSGNARPNNPDW

SEQ ID NO: 678 - protein, 17 aa, Artificial Sequence
  Homo sapiens Fibrinogen alpha chain precursor epitope
FLAEGGGVRGPRVVERH

SEQ ID NO: 679 - protein, 20 aa, Artificial Sequence
  Homo sapiens fibrinogen alpha chain preproprotein, isoform alpha epitope
DHEGTHSTKRGHAKSRPVRG

SEQ ID NO: 680 - protein, 15 aa, Artificial Sequence
  Homo sapiens fibrinogen beta chain epitope
PRKQCSKEDGGGWWY

SEQ ID NO: 681 - protein, 17 aa, Artificial Sequence
  Homo sapiens fibrinogen beta chain, isoform CRA_d epitope
NEEGFFSARGHRPLDKK

SEQ ID NO: 682 - protein, 24 aa, Artificial Sequence
  Homo sapiens fibrinogen beta chain, isoform CRA_i epitope
EEAPSLRPAPPPISGGGYRARPAK

SEQ ID NO: 683 - protein, 6 aa, Artificial Sequence
  Homo sapiens Fibronectin precursor epitope
LTSRPA

SEQ ID NO: 684 - protein, 18 aa, Artificial Sequence
  Homo sapiens filaggrin epitope
DSGHRGYSGSQASDNEGH

SEQ ID NO: 685 - protein, 8 aa, Artificial Sequence
  Homo sapiens Follistatin-related protein 1 epitope
LKFVEQNE

SEQ ID NO: 686 - protein, 10 aa, Artificial Sequence
  Homo sapiens Forkhead box protein E3 epitope
PTPAPGPGRR

SEQ ID NO: 687 - protein, 7 aa, Artificial Sequence
  Homo sapiens GAD65 autoantigen glutamic acid decarboxylase epitope
APAMIPP

SEQ ID NO: 688 - protein, 10 aa, Artificial Sequence
  Triticum aestivum Gamma-gliadin precursor epitope
LQPQQPFPQQ

SEQ ID NO: 689 - protein, 21 aa, Artificial Sequence
  Chironomus thummi thummi Globin CTT-III epitope
AHTDFAGAEAAWGATLDTFFG

SEQ ID NO: 690 - protein, 11 aa, Artificial Sequence
  Chironomus thummi thummi Globin CTT-III precursor epitope
GVTHDQLNNFR

SEQ ID NO: 691 - protein, 23 aa, Artificial Sequence
  Chironomus thummi thummi Globin CTT-IV precursor epitope
KAHTDFAGAEAAWGATLDAFFGM

SEQ ID NO: 692 - protein, 35 aa, Artificial Sequence
  Chironomus thummi thummi Globin CTT-VI precursor epitope
IVSFLSEVISLAGSDANIPAIQNLAKELATSHKPR

SEQ ID NO: 693 - protein, 35 aa, Artificial Sequence
  Chironomus thummi thummi Globin CTT-VIII epitope
IVGFFSEVIGLIGNPENRPALKTLIDGLASSHKAR

SEQ ID NO: 694 - protein, 9 aa, Artificial Sequence
  Hevea brasiliensis Glucan endo-1,3-beta-glucosidase, basic vacuolar isoform epitope
AWLAQFVLP

SEQ ID NO: 695 - protein, 20 aa, Artificial Sequence
  Homo sapiens glutamate decarboxylase epitope
FRERQSSKNLLSCENSDRDA

SEQ ID NO: 696 - protein, 20 aa, Artificial Sequence
  Homo sapiens Glutamate decarboxylase 1 epitope
MASSTPSSSATSSNAGADPN

SEQ ID NO: 697 - protein, 19 aa, Artificial Sequence
  Homo sapiens Glutamate decarboxylase 2 epitope
PGSGFWSFGSEDGSGDSEN

SEQ ID NO: 698 - protein, 15 aa, Artificial Sequence
  Homo sapiens glutamate receptor, ionotropic, N-methyl D-aspartate 2A epitope
SVSYDDWDYSLEARV

SEQ ID NO: 699 - protein, 14 aa, Artificial Sequence
  Homo sapiens glutathione peroxidase-GI epitope
NEHPVFAYLKDKLP

SEQ ID NO: 700 - protein, 14 aa, Artificial Sequence
  Triticum aestivum Glutenin, high molecular weight subunit DX5 epitope
AQGQQPGQGQQGQQ

SEQ ID NO: 701 - protein, 5 aa, Artificial Sequence
  Triticum aestivum Glutenin, high molecular weight subunit DX5 precursor epitope
QQPGQ

SEQ ID NO: 702 - protein, 5 aa, Artificial Sequence
  Triticum aestivum Glutenin, low molecular weight subunit precursor epitope
QQQPP

SEQ ID NO: 703 - protein, 15 aa, Artificial Sequence
  Phaseolus vulgaris Glycine-rich cell wall structural protein 1.8 precursor epitope
GGYGDGGAHGGGYGG

SEQ ID NO: 704 - protein, 15 aa, Artificial Sequence
  Arachis hypogaea Glycinin epitope
ALSRLVLRRNALRRP

SEQ ID NO: 705 - protein, 13 aa, Artificial Sequence
  Glycine max Glycinin G1 precursor epitope
GAIVTVKGGLSVI

SEQ ID NO: 706 - protein, 15 aa, Artificial Sequence
  Glycine max Glycinin G2 precursor epitope
ALSRCTLNRNALRRP

SEQ ID NO: 707 - protein, 15 aa, Artificial Sequence
  Holcus lanatus group V allergen epitope
ANVPPADKYKTFEAA

SEQ ID NO: 708 - protein, 38 aa, Artificial Sequence
  Homo sapiens Gu protein epitope
IDAPKPKKMKKEKEMNGETREKSPKLKNGFPHPEPDCN

SEQ ID NO: 709 - protein, 17 aa, Artificial Sequence
  Homo sapiens H1 histone family, member 0 epitope
KEIKKVATPKKASKPKK

SEQ ID NO: 710 - protein, 12 aa, Artificial Sequence
  Homo sapiens heat shock 60kDa protein 1 (chaperonin) epitope
AYAKDVKFGADA

SEQ ID NO: 711 - protein, 6 aa, Artificial Sequence
  Homo sapiens Heat shock protein HSP 90-beta epitope
GLELPE

SEQ ID NO: 712 - protein, 15 aa, Artificial Sequence
  Homo sapiens high mobility group protein 17 epitope
KKAPAKKGEKVPKGK

SEQ ID NO: 713 - protein, 22 aa, Artificial Sequence
  Homo sapiens High mobility group protein B1 epitope
AKGKPDAAKKGVVKAEKSKKKK

SEQ ID NO: 714 - protein, 15 aa, Artificial Sequence
  Homo sapiens high-mobility group box 2 epitope
FEDMAKSDKARYDRE

SEQ ID NO: 715 - protein, 43 aa, Artificial Sequence
  Homo sapiens histidyl-tRNA synthetase, cytoplasmic epitope
AERAALEELVKLQGERVRGLKQQKASAELIEEEVAKLLKLKAQ

SEQ ID NO: 716 - protein, 16 aa, Artificial Sequence
  Homo sapiens Histone H1.4 epitope
SETAPAAPAAPAPAEK

SEQ ID NO: 717 - protein, 15 aa, Artificial Sequence
  Homo sapiens histone H1b epitope
KPKAAKPKKAAAKKK

SEQ ID NO: 718 - protein, 20 aa, Artificial Sequence
  Homo sapiens Histone H2A.Z epitope
GKAKTKAVSRSQRAGLQFPV

SEQ ID NO: 719 - protein, 15 aa, Artificial Sequence
  Homo sapiens histone H3 epitope
LPFQRLVREIAQDFK

SEQ ID NO: 720 - protein, 10 aa, Artificial Sequence
  Homo sapiens Histone H3-like centromeric protein A epitope
KPEAPRRRSP

SEQ ID NO: 721 - protein, 8 aa, Artificial Sequence
  Homo sapiens HLA class I histocompatibility antigen, B-27 alpha chain precursor epitope
KAKAQTDR

SEQ ID NO: 722 - protein, 16 aa, Artificial Sequence
  Homo sapiens HLA-B27 epitope
AKAQTDREDLRTLLRY

SEQ ID NO: 723 - protein, 20 aa, Artificial Sequence
  Homo sapiens HLA-DR3 epitope
RPDAEYWNSQKDLLEQKRGR

SEQ ID NO: 724 - protein, 15 aa, Artificial Sequence
  Homo sapiens HMG-17 epitope
DGKAKVKDEPQRRSA

SEQ ID NO: 725 - protein, 13 aa, Artificial Sequence
  Homo sapiens HNRNPA2B1 protein epitope
ETTEESLRNYYEQ

SEQ ID NO: 726 - protein, 35 aa, Artificial Sequence
  Homo sapiens hypothetical protein epitope
ANEDAAQGIANWDAVQDIANEDGFHGIDIEDAAQG

SEQ ID NO: 727 - protein, 12 aa, Artificial Sequence
  Oryza sativa Japonica Group hypothetical protein epitope
AFNHFGIQLVQR

SEQ ID NO: 728 - protein, 20 aa, Artificial Sequence
  Homo sapiens Ig alpha-1 chain C region epitope
PVPSTPPTPSPSTPPTPSPS

SEQ ID NO: 729 - protein, 7 aa, Artificial Sequence
  Homo sapiens Ig gamma-1 chain C region epitope
KFNWYVD

SEQ ID NO: 730 - protein, 7 aa, Artificial Sequence
  Homo sapiens Ig gamma-3 chain C region epitope
DGSFFLY

SEQ ID NO: 731 - protein, 7 aa, Artificial Sequence
  Homo sapiens Ig heavy chain V-III region (ART) epitope
CSVMHEG

SEQ ID NO: 732 - protein, 16 aa, Artificial Sequence
  Homo sapiens Ig lambda chain V-II region MGC epitope
SGLQAEDEADYYCSSY

SEQ ID NO: 733 - protein, 7 aa, Artificial Sequence
  Homo sapiens Ig L-chain V-region epitope
APSVTLF

SEQ ID NO: 734 - protein, 7 aa, Artificial Sequence
  Homo sapiens Immunoglobulin heavy chain epitope
DKSRWQE

SEQ ID NO: 735 - protein, 16 aa, Artificial Sequence
  Homo sapiens immunoglobulin light chain epitope
KATLVCLISDFYPGAV

SEQ ID NO: 736 - protein, 7 aa, Artificial Sequence
  Homo sapiens immunoglobulin light chain variable region epitope
AGEKVTM

SEQ ID NO: 737 - protein, 3 aa, Artificial Sequence
  Homo sapiens Insulin precursor epitope
TSI

SEQ ID NO: 738 - protein, 14 aa, Artificial Sequence
  Homo sapiens Integrin alpha-6 epitope
LKRDMKSAHLLPEH

SEQ ID NO: 739 - protein, 18 aa, Artificial Sequence
  Homo sapiens Integrin beta-3 precursor epitope
CAPESIEFPVSEARVLED

SEQ ID NO: 740 - protein, 14 aa, Artificial Sequence
  Homo sapiens interferon alpha 2 epitope
CDLPQTHSLGSRRT

SEQ ID NO: 741 - protein, 14 aa, Artificial Sequence
  Homo sapiens interferon alpha A epitope
EDSILAVRKYFQRI

SEQ ID NO: 742 - protein, 12 aa, Artificial Sequence
  Homo sapiens interferon beta precursor epitope
HLKRYYGRILHY

SEQ ID NO: 743 - protein, 14 aa, Artificial Sequence
  Homo sapiens interferon-alpha 2 epitope
LMLLAQMRRISLFS

SEQ ID NO: 744 - protein, 37 aa, Artificial Sequence
  Homo sapiens Islet amyloid polypeptide precursor epitope
MGILKLQVFLIVLSVALNHLKATPIESHQVEKRKCNT

SEQ ID NO: 745 - protein, 14 aa, Artificial Sequence
  Bos taurus Kappa-casein precursor epitope
AKYIPIQYVLSRYP

SEQ ID NO: 746 - protein, 10 aa, Artificial Sequence
  Homo sapiens Ku antigen epitope
RGDGPFRLGG

SEQ ID NO: 747 - protein, 15 aa, Artificial Sequence
  Homo sapiens leukotriene B4 receptor 2 epitope
GRGNGDPGGGMEKDG

SEQ ID NO: 748 - protein, 14 aa, Artificial Sequence
  Homo sapiens liver histone H1e epitope
IKKVATPKKASPKK

SEQ ID NO: 749 - protein, 23 aa, Artificial Sequence
  Homo sapiens Lupus La protein epitope
AQPGSGKGKVQFQGKKTKFASDD

SEQ ID NO: 750 - protein, 30 aa, Artificial Sequence
  Homo sapiens lymphocyte activation gene 3 protein precursor epitope
GPPAAAPGHPLAPGPHPAAPSSWGPRPRRY

SEQ ID NO: 751 - protein, 10 aa, Artificial Sequence
  Homo sapiens m3 muscarinic cholinergic receptor epitope
EPTITFGTAI

SEQ ID NO: 752 - protein, 20 aa, Artificial Sequence
  Alternaria alternata Major allergen Alt a 1 precursor epitope
ADPVTTEGDYVVKISEFYGR

SEQ ID NO: 753 - protein, 15 aa, Artificial Sequence
  Anisakis simplex Major allergen Ani s 1 epitope
CKMPDRGACALGKKP

SEQ ID NO: 754 - protein, 13 aa, Artificial Sequence
  Aspergillus fumigatus Major allergen Asp f 1 epitope
LNPKTNKWEDKRY

SEQ ID NO: 755 - protein, 10 aa, Artificial Sequence
  Aspergillus fumigatus Major allergen Asp f 2 epitope
AHILRWGNES

SEQ ID NO: 756 - protein, 20 aa, Artificial Sequence
  Bos taurus major allergen beta-lactoglobulin epitope
LQKWENDECAQKKIIAEKTK

SEQ ID NO: 757 - protein, 14 aa, Artificial Sequence
  Felis catus Major allergen I polypeptide chain 1 precursor epitope
DAKMTEEDKENALS

SEQ ID NO: 758 - protein, 14 aa, Artificial Sequence
  Felis catus Major allergen I polypeptide chain 2 precursor epitope
EPERTAMKKIQDCY

SEQ ID NO: 759 - protein, 11 aa, Artificial Sequence
  Felis catus major allergen I, polypeptide chain 1 epitope
LLDKIYTSPLC

SEQ ID NO: 760 - protein, 29 aa, Artificial Sequence
  Turbo cornutus major allergen Tur c1 - Turbo cornutus epitope
LEDELLAEKEKYKAISDELDQTFAELAGY

SEQ ID NO: 761 - protein, 25 aa, Artificial Sequence
  Dermatophagoides pteronyssinus major house dust allergen epitope
LAHRNQSLDLAEQELVDCASQHGCH

SEQ ID NO: 762 - protein, 9 aa, Artificial Sequence
  Hevea brasiliensis Major latex allergen Hev b 5 epitope
APPASEQET

SEQ ID NO: 763 - protein, 43 aa, Artificial Sequence
  Dermatophagoides pteronyssinus Major mite fecal allergen Der p 1 epitope
AREQSCRRPNAQRFGISNYCQIYPPNANKIREALAQPQRYCRH

SEQ ID NO: 764 - protein, 12 aa, Artificial Sequence
  Olea europaea Major pollen allergen epitope
FTEVGYTRAEGL

SEQ ID NO: 765 - protein, 10 aa, Artificial Sequence
  Betula pendula Major pollen allergen Bet v 1-A epitope
DGDNLFPKVA

SEQ ID NO: 766 - protein, 11 aa, Artificial Sequence
  Chamaecyparis obtusa Major pollen allergen Cha o 1 precursor epitope
WRSTQDSFNNG

SEQ ID NO: 767 - protein, 17 aa, Artificial Sequence
  Corylus avellana Major pollen allergen Cor a 1 epitope
YVLDGDKLLPKVAPQAL

SEQ ID NO: 768 - protein, 27 aa, Artificial Sequence
  Holcus lanatus Major pollen allergen Hol l 1 precursor epitope
AKSTWYGKPTGAGPKDNGGACGYKDVD

SEQ ID NO: 769 - protein, 12 aa, Artificial Sequence
  Juniperus ashei Major pollen allergen Jun a 1 precursor epitope
AFNQFGPNAGQR

SEQ ID NO: 770 - protein, 34 aa, Artificial Sequence
  Olea europaea major pollen allergen Ole e 1 epitope
SGRKDCNEIPTEGWVKPSLKFILNTVNGTTRTVN

SEQ ID NO: 771 - protein, 9 aa, Artificial Sequence
  Malus x domestica mal d 3 epitope
RTTADRQTA

SEQ ID NO: 772 - protein, 15 aa, Artificial Sequence
  Homo sapiens MBP protein epitope
ENPVVHFFKNIVTPR

SEQ ID NO: 773 - protein, 30 aa, Artificial Sequence
  Homo sapiens melanin-concentrating hormone receptor 1, isoform CRA_a epitope
AEHASRMSVLRAKPMSNSQRLLLLSPGSPP

SEQ ID NO: 774 - protein, 16 aa, Artificial Sequence
  Homo sapiens Melanocyte protein Pmel 17 precursor epitope
QVPTTEVVGTTPGQAP

SEQ ID NO: 775 - protein, 6 aa, Artificial Sequence
  Homo sapiens MHC classII HLA-DRB1 epitope
EQRRAA

SEQ ID NO: 776 - protein, 20 aa, Artificial Sequence
  Homo sapiens MHC HLA-DR1-beta epitope
RPDAEYWNSQKDLLEQRRAA

SEQ ID NO: 777 - protein, 16 aa, Artificial Sequence
  Blomia tropicalis Mite allergen Blo t 5 epitope
EEAQTLSKILLKDLKE

SEQ ID NO: 778 - protein, 5 aa, Artificial Sequence
  Dermatophagoides farinae Mite group 2 allergen Der f 2 precursor epitope
DPCII

SEQ ID NO: 779 - protein, 15 aa, Artificial Sequence
  Dermatophagoides pteronyssinus Mite group 2 allergen Der p 2 precursor epitope
DQVDVKDCANHEIKK

SEQ ID NO: 780 - protein, 33 aa, Artificial Sequence
  Lepidoglyphus destructor Mite group 2 allergen Lep d 2 precursor epitope
AANQDTAKVTIKVLAKVAGTTIQVPGLETDGCK

SEQ ID NO: 781 - protein, 6 aa, Artificial Sequence
  Triticum aestivum monomeric alpha-amylase inhibitor epitope
AASVPE

SEQ ID NO: 782 - protein, 21 aa, Artificial Sequence
  Homo sapiens Muscarinic acetylcholine receptor M1 epitope
QYLVGERTVLAGQCYIQFLSQ

SEQ ID NO: 783 - protein, 17 aa, Artificial Sequence
  Homo sapiens myelin associated glycoprotein epitope
DSYTLTEELAYAEIRVK

SEQ ID NO: 784 - protein, 13 aa, Artificial Sequence
  Homo sapiens Myelin basic protein epitope
IVTPRTPPPSQGK

SEQ ID NO: 785 - protein, 26 aa, Artificial Sequence
  Homo sapiens myelin oligodendrocyte glycoprotein epitope
ALVGDEVELPCRISPGKNATGMELGW

SEQ ID NO: 786 - protein, 5 aa, Artificial Sequence
  Homo sapiens myelin oligodendrocyte glycoprotein isoform alpha6 precursor epitope
HRTFE

SEQ ID NO: 787 - protein, 5 aa, Artificial Sequence
  Homo sapiens myelin proteolipid protein epitope
ADARM

SEQ ID NO: 788 - protein, 21 aa, Artificial Sequence
  Homo sapiens Myelin-associated glycoprotein precursor epitope
GHWGAWMPSSISAFEGTCVSI

SEQ ID NO: 789 - protein, 26 aa, Artificial Sequence
  Homo sapiens Myelin-oligodendrocyte glycoprotein precursor epitope
GQFRVIGPRHPIRALVGDEVELPCRI

SEQ ID NO: 790 - protein, 8 aa, Artificial Sequence
  Homo sapiens Myeloblastin precursor epitope
AHRPPSPA

SEQ ID NO: 791 - protein, 10 aa, Artificial Sequence
  Homo sapiens Myeloperoxidase epitope
GSASPMELLS

SEQ ID NO: 792 - protein, 20 aa, Artificial Sequence
  Homo sapiens Myosin-11 epitope
ALKTELEDTLDSTATQQELR

SEQ ID NO: 793 - protein, 8 aa, Artificial Sequence
  Homo sapiens Neurofilament heavy polypeptide (NF-H) (Neurofilament triplet H protein) (200 kDa neurofilament protein) epitope
AKSPEKAK

SEQ ID NO: 794 - protein, 16 aa, Artificial Sequence
  Homo sapiens nicotinic acetylcholine receptor alpha subunit|AChR alpha subunit epitope
EVNQIVTTNVRLKQQW

SEQ ID NO: 795 - protein, 10 aa, Artificial Sequence
  Homo sapiens Non-histone chromosomal protein HMG-17 epitope
VKDEPQRRSA

SEQ ID NO: 796 - protein, 9 aa, Artificial Sequence
  Prunus armeniaca Non-specific lipid-transfer protein 1 epitope
VNPNNAAAL

SEQ ID NO: 797 - protein, 15 aa, Artificial Sequence
  Prunus armeniaca Non-specific lipid-transfer protein 1 (LTP 1) (Major allergen Pru ar 3) epitope
LARTTPDRRTACNCL

SEQ ID NO: 798 - protein, 18 aa, Artificial Sequence
  Prunus domestica Non-specific lipid-transfer protein 1 (LTP 1) (Major allergen Pru d 3) epitope
LARTTADRRAACNCLKQL

SEQ ID NO: 799 - protein, 15 aa, Artificial Sequence
  Malus x domestica Non-specific lipid-transfer protein precursor (LTP) (Allergen Mal d 3) epitope
ADRQTACNCLKNLAG

SEQ ID NO: 800 - protein, 10 aa, Artificial Sequence
  Homo sapiens NR2 subunit NMDA receptor epitope
DWEYSVWLSN

SEQ ID NO: 801 - protein, 8 aa, Artificial Sequence
  Homo sapiens nuclear autoantigen Sp-100 isoform 1 epitope
EVFISAPR

SEQ ID NO: 802 - protein, 12 aa, Artificial Sequence
  Olea europaea Ole e 1 protein epitope
EDVPQPPVSQFH

SEQ ID NO: 803 - protein, 25 aa, Artificial Sequence
  Olea europaea Ole e 1.0102 protein epitope
EDVPQPPVSQFHIQGQVYCDTCRAG

SEQ ID NO: 804 - protein, 10 aa, Artificial Sequence
  Triticum aestivum Omega gliadin storage protein epitope
QQPQQSFPQQ

SEQ ID NO: 805 - protein, 7 aa, Artificial Sequence
  Triticum aestivum omega-5 gliadin epitope
QQFHQQQ

SEQ ID NO: 806 - protein, 35 aa, Artificial Sequence
  Aspergillus fumigatus Oryzin precursor epitope
ASNTSPASAPNALTVAAINKSNARASFSNYGSVVD

SEQ ID NO: 807 - protein, 9 aa, Artificial Sequence
  Gallus gallus Ovalbumin epitope
CFDVFKELK

SEQ ID NO: 808 - protein, 10 aa, Artificial Sequence
  Gallus gallus Ovomucoid epitope
CNFCNAVVES

SEQ ID NO: 809 - protein, 14 aa, Artificial Sequence
  Gallus gallus Ovomucoid precursor epitope
AEVDCSRFPNATDK

SEQ ID NO: 810 - protein, 10 aa, Artificial Sequence
  Glycine max P34 probable thiol protease precursor epitope
ASWDWRKKGV

SEQ ID NO: 811 - protein, 10 aa, Artificial Sequence
  Glycine max P34 probable thiol protease precursor; Gly m 1 epitope
PQEFSKKTYQ

SEQ ID NO: 812 - protein, 9 aa, Artificial Sequence
  Homo sapiens p70 autoantigen epitope
EALTKHFQD

SEQ ID NO: 813 - protein, 20 aa, Artificial Sequence
  Homo sapiens PADI-H protein epitope
KAASGSTGDQKVQISYYGPK

SEQ ID NO: 814 - protein, 9 aa, Artificial Sequence
  Parietaria judaica Par j epitope
GTSSCRLVP

SEQ ID NO: 815 - protein, 47 aa, Artificial Sequence
  Blomia tropicalis Paramyosin epitope
EKLRDQKEALARENKKLADDLAEAKSQLNDAHRRIHEQEIEIKRLEN

SEQ ID NO: 816 - protein, 8 aa, Artificial Sequence
  Gadus morhua callarias Parvalbumin beta epitope
AAEAACFK

SEQ ID NO: 817 - protein, 15 aa, Artificial Sequence
  Salmo salar parvalbumin like 1 epitope
ADIKTALEARKAADT

SEQ ID NO: 818 - protein, 12 aa, Artificial Sequence
  Juniperus ashei Pathogenesis-related protein precursor epitope
ADINAVCPSELK

SEQ ID NO: 819 - protein, 12 aa, Artificial Sequence
  Nicotiana tabacum Pectate lyase epitope
AYNHFGKRLDQR

SEQ ID NO: 820 - protein, 12 aa, Artificial Sequence
  Musa acuminata AAA Group pectate lyase 2 epitope
AFNHFGEGLIQR

SEQ ID NO: 821 - protein, 15 aa, Artificial Sequence
  Farfantepenaeus aztecus Pen a 1 allergen epitope
ANIQLVEKDKALSNA

SEQ ID NO: 822 - protein, 43 aa, Artificial Sequence
  Dermatophagoides pteronyssinus Peptidase 1 precursor (Major mite fecal allergen Der p 1) (Allergen Der p I) epitope
AREQSCRRPNAQRFGISNYCQIYPPNVNKIREALAQTHSAIAV

SEQ ID NO: 823 - protein, 3 aa, Artificial Sequence
  Homo sapiens pericentriolar material 1 protein epitope
KDC

SEQ ID NO: 824 - protein, 20 aa, Artificial Sequence
  Homo sapiens Periplakin epitope
IHDRKSGKKFSIEEALQSGR

SEQ ID NO: 825 - protein, 45 aa, Artificial Sequence
  Apis mellifera Phospholipase A2 precursor epitope
LIDTKCYKLEHPVTGCGERTEGRCLHYTVDKSKPKVYQWFDLRKY

SEQ ID NO: 826 - protein, 14 aa, Artificial Sequence
  Myrmecia pilosula Pilosulin-1 precursor (Major allergen Myr p 1) (Myr p I) epitope
KEAIPMAVEMAKSQ

SEQ ID NO: 827 - protein, 8 aa, Artificial Sequence
  Homo sapiens plasma protease C1 inhibitor precursor epitope
ASAISVAR

SEQ ID NO: 828 - protein, 6 aa, Artificial Sequence
  Homo sapiens platelet glycoprotein IIIa epitope
RARAKW

SEQ ID NO: 829 - protein, 12 aa, Artificial Sequence
  Homo sapiens plexin domain containing 1, isoform CRA_b epitope
NCSWCHVLQRCS

SEQ ID NO: 830 - protein, 15 aa, Artificial Sequence
  Homo sapiens PM/Scl 100kD nucleolar protein epitope
CIAAKKIKQSVGNKS

SEQ ID NO: 831 - protein, 8 aa, Artificial Sequence
  Betula pendula Polcalcin Bet v 4 epitope
FGRANRGL

SEQ ID NO: 832 - protein, 36 aa, Artificial Sequence
  Phleum pratense Polcalcin Phl p 7 (Calcium-binding pollen allergen Phl p 7) (P7) epitope
ADDMERIFKRFDTNGDGKISLSELTDALRTLGSTSA

SEQ ID NO: 833 - protein, 25 aa, Artificial Sequence
  Lolium perenne pollen allergen epitope
EGGTKSEVEDVIPEGWKADTSYSAK

SEQ ID NO: 834 - protein, 12 aa, Artificial Sequence
  Ambrosia artemisiifolia Pollen allergen Amb a 1.4 epitope
AFNKFTDNVDQR

SEQ ID NO: 835 - protein, 8 aa, Artificial Sequence
  Ambrosia artemisiifolia Pollen allergen Amb a 2 precursor epitope
MPRCRFGF

SEQ ID NO: 836 - protein, 15 aa, Artificial Sequence
  Ambrosia artemisiifolia var. elatior Pollen allergen Amb a 3 epitope
CDIKDPIRLEPGGPD

SEQ ID NO: 837 - protein, 31 aa, Artificial Sequence
  Betula pendula pollen allergen Bet v 1 epitope
KAEQVKASKEMGETLLRAVESYLLAHSDAYN

SEQ ID NO: 838 - protein, 20 aa, Artificial Sequence
  Poa pratensis Pollen allergen KBG 60 precursor epitope
AANKYKTFVATFGAASNKAF

SEQ ID NO: 839 - protein, 25 aa, Artificial Sequence
  Lolium perenne Pollen allergen Lol p 2-A (Lol p II-A) epitope
EKGMRNVFDDVVPADFKVGTTYKPE

SEQ ID NO: 840 - protein, 27 aa, Artificial Sequence
  Lolium perenne Pollen allergen Lol p 3 (Lol p III) epitope
KGGMKNVFDEVIPTAFTVGKTYTPEYN

SEQ ID NO: 841 - protein, 12 aa, Artificial Sequence
  Lolium perenne Pollen allergen Lol p VA precursor epitope
AAEGATPEAKYD

SEQ ID NO: 842 - protein, 15 aa, Artificial Sequence
  Phleum pratense Pollen allergen Phl p 1 precursor epitope
APYHFDLSGHAFGAM

SEQ ID NO: 843 - protein, 8 aa, Artificial Sequence
  Zea mays pollen allergen Phl p 11 epitope
RDRARVPL

SEQ ID NO: 844 - protein, 12 aa, Artificial Sequence
  Phleum pratense pollen allergen Phl pI epitope
IPKVPPGPNITA

SEQ ID NO: 845 - protein, 20 aa, Artificial Sequence
  Cryptomeria japonica Polygalacturonase precursor epitope
GQCKWVNGREICNDRDRPTA

SEQ ID NO: 846 - protein, 30 aa, Artificial Sequence
  Parietaria judaica Probable non-specific lipid-transfer protein epitope
QETCGTMVRALMPCLPFVQGKEKEPSKGCC

SEQ ID NO: 847 - protein, 10 aa, Artificial Sequence
  Parietaria judaica Probable non-specific lipid-transfer protein 2 epitope
AEVPKKCDIK

SEQ ID NO: 848 - protein, 30 aa, Artificial Sequence
  Parietaria judaica Probable non-specific lipid-transfer protein 2 precursor epitope
EACGKVVQDIMPCLHFVKGEEKEPSKECCS

SEQ ID NO: 849 - protein, 12 aa, Artificial Sequence
  Solanum lycopersicum Probable pectate lyase P59 epitope
AFNHFGKRLIQR

SEQ ID NO: 850 - protein, 11 aa, Artificial Sequence
  Homo sapiens profilaggrin epitope
GGQGSRHQQAR

SEQ ID NO: 851 - protein, 10 aa, Artificial Sequence
  Cucumis melo profilin epitope
AFRLEEIAAI

SEQ ID NO: 852 - protein, 56 aa, Artificial Sequence
  Glycine max Profilin-1 epitope
WAQSTDFPQFKPEEITAIMNDFNEPGSLAPTGLYLGGTKYMVIQGEPGAVIRGKKG

SEQ ID NO: 853 - protein, 43 aa, Artificial Sequence; identical to SEQ ID NO: 491
  Hevea brasiliensis Pro-hevein precursor epitope

SEQ ID NO: 854 - protein, 15 aa, Artificial Sequence
  Homo sapiens Proliferating cell nuclear antigen epitope
LKYYLAPKIEDEEGS

SEQ ID NO: 855 - protein, 9 aa, Artificial Sequence
  Homo sapiens Proline-rich transmembrane protein 2 epitope
HSEAETGPP

SEQ ID NO: 856 - protein, 15 aa, Artificial Sequence
  Homo sapiens proteasome (prosome, macropain) activator subunit 3 (PA28 gamma; Ki), isoform CRA_a epitope
LDGPTYKRRLDECEE

SEQ ID NO: 857 - protein, 13 aa, Artificial Sequence
  Homo sapiens protein tyrosine phosphatase-like autoantigen epitope
GAHGDTTPEYQDL

SEQ ID NO: 858 - protein, 20 aa, Artificial Sequence
  Homo sapiens protein-arginine deiminase type-4 epitope
AFFPNMVNMLVLGKHLGIPK

SEQ ID NO: 859 - protein, 15 aa, Artificial Sequence
  Homo sapiens proteinase 3 epitope
CATRLFPDFFTRVAL

SEQ ID NO: 860 - protein, 10 aa, Artificial Sequence
  Prunus persica pru p 1 epitope
GKCGVSIPYK

SEQ ID NO: 861 - protein, 15 aa, Artificial Sequence
  Prunus dulcis prunin 1 precursor epitope
EESQQSSQQGRQQEQ

SEQ ID NO: 862 - protein, 15 aa, Artificial Sequence
  Prunus dulcis prunin 2 precursor epitope
DSQPQQFQQQQQQQQ

SEQ ID NO: 863 - protein, 11 aa, Artificial Sequence
  Hesperocyparis arizonica putative allergen Cup a 1 epitope
WRFTRDAFTNG

SEQ ID NO: 864 - protein, 11 aa, Artificial Sequence
  Homo sapiens Putative HTLV-1-related endogenous sequence (p25) epitope
PTRAPSGPRPP

SEQ ID NO: 865 - protein, 8 aa, Artificial Sequence
  Homo sapiens Putative small nuclear ribonucleoprotein polypeptide E-like protein 1 epitope
EIHSKTKS

SEQ ID NO: 866 - protein, 18 aa, Artificial Sequence
  Homo sapiens Receptor tyrosine-protein kinase erbB-2 precursor epitope
PESFDGDPASNTAPLQPE

SEQ ID NO: 867 - protein, 13 aa, Artificial Sequence
  Homo sapiens Receptor-type tyrosine-protein phosphatase-like N precursor epitope
KERLAALGPEGAH

SEQ ID NO: 868 - protein, 11 aa, Artificial Sequence
  Homo sapiens recombinant IgG2 heavy chain epitope
EPQVVTLPPSR

SEQ ID NO: 869 - protein, 20 aa, Artificial Sequence
  Homo sapiens Replication protein A 32 kDa subunit epitope
RSFQNKKSLVAFKIMPLEDM

SEQ ID NO: 870 - protein, 10 aa, Artificial Sequence
  Aspergillus fumigatus Ribonuclease mitogillin precursor epitope
FPTFPDGHDY

SEQ ID NO: 871 - protein, 23 aa, Artificial Sequence
  Homo sapiens ribosomal protein L7 epitope
ELKIKRLRKKFAQKMLRKARRKL

SEQ ID NO: 872 - protein, 14 aa, Artificial Sequence
  Homo sapiens ribosomal protein P2 epitope
SEESDDDMGFGLFD

SEQ ID NO: 873 - protein, 12 aa, Artificial Sequence
  Mangifera indica ripening-related pectate lyase epitope
AYNHFGEGLIQR

SEQ ID NO: 874 - protein, 21 aa, Artificial Sequence
  Homo sapiens RNA binding protein, autoantigenic (hnRNP-associated with lethal yellow homolog (mouse)), isoform CRA_c epitope
GGGGGGSGGGGSGGGGGGGSS

SEQ ID NO: 875 - protein, 21 aa, Artificial Sequence
  Homo sapiens Ro ribonucleoprotein epitope
DGYVWQVTDMNRLHRFLCFGS

SEQ ID NO: 876 - protein, 10 aa, Artificial Sequence
  Hevea brasiliensis Rubber elongation factor protein epitope
AEDEDNQQGQ

SEQ ID NO: 877 - protein, 14 aa, Artificial Sequence
  Homo sapiens S-arrestin epitope
FLGELTSSEVATEV

SEQ ID NO: 878 - protein, 15 aa, Artificial Sequence
  Juglans regia seed storage protein epitope
DDNGLEETICTLRLR

SEQ ID NO: 879 - protein, 15 aa, Artificial Sequence
  Arachis hypogaea seed storage protein SSP2 epitope
CGLRAPQRCDLDVES

SEQ ID NO: 880 - protein, 8 aa, Artificial Sequence
  Gallus gallus serine (or cysteine) proteinase inhibitor, clade B (ovalbumin), member 3 epitope
RPNATYSL

SEQ ID NO: 881 - protein, 8 aa, Artificial Sequence
  Gallus gallus Serum albumin epitope
QSRATLGI

SEQ ID NO: 882 - protein, 17 aa, Artificial Sequence
  Bos taurus Serum albumin precursor epitope
DDSPDLPKLKPDPNTLC

SEQ ID NO: 883 - protein, 8 aa, Artificial Sequence
  Homo sapiens small nuclear ribonucleoprotein epitope
PPPGIRGP

SEQ ID NO: 884 - protein, 8 aa, Artificial Sequence
  Homo sapiens small nuclear ribonucleoprotein B' epitope
PPPGMRGP

SEQ ID NO: 885 - protein, 24 aa, Artificial Sequence
  Homo sapiens small nuclear ribonucleoprotein D1 polypeptide epitope
KMTLKNREPVQLETLSIRGNRIRY

SEQ ID NO: 886 - protein, 23 aa, Artificial Sequence
  Homo sapiens small nuclear ribonucleoprotein D2 isoform 1 epitope
GKKKSKPVNKDRYISKMFLRGDS

SEQ ID NO: 887 - protein, 8 aa, Artificial Sequence
  Homo sapiens small nuclear ribonucleoprotein F epitope
EEEEDGEM

SEQ ID NO: 888 - protein, 8 aa, Artificial Sequence
  Homo sapiens small nuclear ribonucleoprotein G epitope
WSKAHPPE

SEQ ID NO: 889 - protein, 9 aa, Artificial Sequence
  Homo sapiens small nuclear ribonucleoprotein polypeptide A epitope
AMKISFAKK

SEQ ID NO: 890 - protein, 7 aa, Artificial Sequence
  Homo sapiens small nuclear ribonucleoprotein polypeptide B epitope
PPGMRPP

SEQ ID NO: 891 - protein, 12 aa, Artificial Sequence
  Homo sapiens small nuclear ribonucleoprotein polypeptide B/B' isoform B epitope
MGRGAPPPGMMG

SEQ ID NO: 892 - protein, 7 aa, Artificial Sequence
  Homo sapiens small nuclear ribonucleoprotein polypeptide C, isoform CRA_b epitope
APGMRPP

SEQ ID NO: 893 - protein, 15 aa, Artificial Sequence
  Homo sapiens small nuclear ribonucleoprotein polypeptide D3 epitope
AARGRGRGMGRGNIF

SEQ ID NO: 894 - protein, 12 aa, Artificial Sequence
  Homo sapiens small nuclear ribonucleoprotein polypeptide N variant epitope
VGRATPPPGIMA

SEQ ID NO: 895 - protein, 23 aa, Artificial Sequence
  Homo sapiens Small nuclear ribonucleoprotein Sm D1 epitope
GRGRGRGRGRGRGRGRGRGGPRR

SEQ ID NO: 896 - protein, 8 aa, Artificial Sequence
  Homo sapiens Small nuclear ribonucleoprotein Sm D2 epitope
EELQKREE

SEQ ID NO: 897 - protein, 8 aa, Artificial Sequence
  Homo sapiens Small nuclear ribonucleoprotein-associated proteins B and B' epitope
RGVGGPSQ

SEQ ID NO: 898 - protein, 10 aa, Artificial Sequence
  Hevea brasiliensis Small rubber particle protein epitope
AEEVEEERLK

SEQ ID NO: 899 - protein, 20 aa, Artificial Sequence
  Homo sapiens Smoothelin epitope
GSTMMQTKTFSSSSSSKKMG

SEQ ID NO: 900 - protein, 15 aa, Artificial Sequence
  Homo sapiens snRNP polypeptide B epitope
PPGMRPPMGPMGIPP

SEQ ID NO: 901 - protein, 14 aa, Artificial Sequence
  Homo sapiens spectrin, alpha, non-erythrocytic 1 (alpha-fodrin), isoform CRA_e epitope
FQFFQRDAEELEKW

SEQ ID NO: 902 - protein, 43 aa, Artificial Sequence
  Homo sapiens steroid 17-alpha-hydroxylase/17,20 lyase epitope
EVPDDGQLPSLEGIPKVVFLIDSFKVKIKVRQAWREAQAEGST

SEQ ID NO: 903 - protein, 15 aa, Artificial Sequence
  Homo sapiens Sucrase-isomaltase, intestinal epitope
DFTYDQVAFNGLPQF

SEQ ID NO: 904 - protein, 12 aa, Artificial Sequence
  Cryptomeria japonica Sugi basic protein precursor epitope
DALTLRTATNIW

SEQ ID NO: 905 - protein, 48 aa, Artificial Sequence
  Aspergillus fumigatus Superoxide dismutase epitope
YTLPPLPYPYDALQPYISQQIMELHHKKHHQTYVNGLNAALEAQKKAA

SEQ ID NO: 906 - protein, 11 aa, Artificial Sequence
  Homo sapiens T cell receptor beta variable 20 epitope
RSLDFQATTMF

SEQ ID NO: 907 - protein, 18 aa, Artificial Sequence
  Homo sapiens T cell receptor beta variable 5 epitope
ALGQGPQFIFQYYEEEER

SEQ ID NO: 908 - protein, 15 aa, Artificial Sequence
  Homo sapiens Tax1-binding protein 1 epitope
EFKKRFSDATSKAHQ

SEQ ID NO: 909 - protein, 16 aa, Artificial Sequence
  Homo sapiens T-cell receptor beta chain epitope
QPLKEQPALNDSRYCL

SEQ ID NO: 910 - protein, 16 aa, Artificial Sequence
  Homo sapiens T-cell receptor beta chain C region epitope
SATFWQNPRNHFRCQV

SEQ ID NO: 911 - protein, 16 aa, Artificial Sequence
  Homo sapiens T-cell receptor beta chain V region YT35 epitope
CKPISGHNSLFWYRQT

SEQ ID NO: 912 - protein, 10 aa, Artificial Sequence
  Homo sapiens T-cell receptor beta-chain (V1-D-J-C) precursor epitope
SPRSGDLSVY

SEQ ID NO: 913 - protein, 21 aa, Artificial Sequence
  Homo sapiens TCR V-beta 6.1 epitope
LGQGPEFLIYFQGTGAADDSG

SEQ ID NO: 914 - protein, 10 aa, Artificial Sequence
  Homo sapiens TCR V-beta 6.3 epitope
DPISGHVSLF

SEQ ID NO: 915 - protein, 20 aa, Artificial Sequence
  Homo sapiens Thyroglobulin epitope
PPARALKRSLWVEVDLLIGS

SEQ ID NO: 916 - protein, 19 aa, Artificial Sequence
  Homo sapiens Thyroid peroxidase epitope
GLPRLETPADLSTAIASRS

SEQ ID NO: 917 - protein, 15 aa, Artificial Sequence
  Homo sapiens thyroid stimulating hormone receptor epitope
EIIGFGQELKNPQEE

SEQ ID NO: 918 - protein, 16 aa, Artificial Sequence
  Homo sapiens thyroid stimulating hormone receptor variant epitope
EEQEDEIIGFGQELKN

SEQ ID NO: 919 - protein, 20 aa, Artificial Sequence
  Homo sapiens Thyrotropin receptor epitope
GQELKNPQEETLQAFDSHYD

SEQ ID NO: 920 - protein, 15 aa, Artificial Sequence
  Homo sapiens transaldolase 1 epitope
AAAQMPAYQELVEEA

SEQ ID NO: 921 - protein, 20 aa, Artificial Sequence
  Trichophyton rubrum Tri r 2 allergen epitope
DCNGHGTHVAGTVGGTKYGL

SEQ ID NO: 922 - protein, 15 aa, Artificial Sequence
  Homo sapiens trinucleotide repeat containing 6A, isoform CRA_b epitope
AFLSVDHLGGGGESM

SEQ ID NO: 923 - protein, 15 aa, Artificial Sequence
  Homo sapiens trinucleotide repeat containing 6A, isoform CRA_c epitope
WGSSSVGPQALSKSG

SEQ ID NO: 924 - protein, 36 aa, Artificial Sequence
  Homo sapiens tripartite motif-containing 67 epitope
LGGGAGGGGDHADKLSLYSETDSGYGSYTPSLKSPN

SEQ ID NO: 925 - protein, 10 aa, Artificial Sequence
  Triticum aestivum Triticum aestivum proteins epitope
LPQQQIPQQP

SEQ ID NO: 926 - protein, 9 aa, Artificial Sequence
  Penaeus tropomyosin epitope
FLAEEADRK

SEQ ID NO: 927 - protein, 20 aa, Artificial Sequence
  Homo sapiens TSHR protein epitope
CHQEEDFRVTCKDIQRIPSL

SEQ ID NO: 928 - protein, 14 aa, Artificial Sequence
  Homo sapiens tubulin beta-6 chain epitope
AACDPRHGRYLTVA

SEQ ID NO: 929 - protein, 10 aa, Artificial Sequence
  Homo sapiens tumor necrosis factor ligand superfamily member 6 epitope
EWEDTYGIVL

SEQ ID NO: 930 - protein, 20 aa, Artificial Sequence
  Paralichthys olivaceus type 1 collagen alpha 2 epitope
MKGLRGHPGLQGMPGPSGPS

SEQ ID NO: 931 - protein, 10 aa, Artificial Sequence
  Triticum aestivum type 1 non-specific lipid transfer protein precursor epitope
ARGTPLKCGV

SEQ ID NO: 932 - protein, 5 aa, Artificial Sequence
  Homo sapiens U1 small nuclear ribonucleoprotein 70 kDa epitope
ERKRR

SEQ ID NO: 933 - protein, 26 aa, Artificial Sequence
  Homo sapiens U1 small nuclear ribonucleoprotein A epitope
AGAARDALQGFKITQNNAMKISFAKK

SEQ ID NO: 934 - protein, 8 aa, Artificial Sequence
  Homo sapiens U1 small nuclear ribonucleoprotein C epitope
PAPGMRPP

SEQ ID NO: 935 - protein, 18 aa, Artificial Sequence
  Anisakis simplex UA3-recognized allergen epitope
MCQCVQKYGTEFCKKRLA

SEQ ID NO: 936 - protein, 9 aa, Artificial Sequence
  Homo sapiens unnamed protein product epitope
AFQQGKIPP

SEQ ID NO: 937 - protein, 8 aa, Artificial Sequence
  Juglans nigra vicilin seed storage protein epitope
SFEDQGRR

SEQ ID NO: 938 - protein, 15 aa, Artificial Sequence
  Anacardium occidentale Vicilin-like protein epitope
AIMGPPTKFSFSLFL

SEQ ID NO: 939 - protein, 10 aa, Artificial Sequence
  Juglans regia vicilin-like protein precursor epitope
DQRSQEERER

SEQ ID NO: 940 - protein, 20 aa, Artificial Sequence
  Homo sapiens Vimentin epitope
RLRSSVPGVRLLQDSVDFSL

SEQ ID NO: 941 - protein, 15 aa, Artificial Sequence
  Homo sapiens von Willebrand factor epitope
HCQICHCDVVNLTCE

SEQ ID NO: 942 - protein, 45 aa, Artificial Sequence
  Homo sapiens von Willebrand factor-cleaving protease precursor epitope
PSHFQQSCLQALEPQAVSSYLSPGAPLKGRPPSPGFQRQRQRQRR

SEQ ID NO: 943 - protein, 15 aa, Artificial Sequence
  Homo sapiens XRCC4 protein epitope
VSKDDSIISSLDVTD

SEQ ID NO: 944 - protein, 8 aa, Artificial Sequence
  OVA epitope
SIINFEKL